European Patent Application EP 4 397 748 A1, published July 10, 2024. Title: Gene sequence construct for gene therapy for HIV infection. Applicant: Kanglin Biotechnology (Hangzhou) Co. Ltd. The sequence listing filed with the application follows.

SEQUENCE LISTING (29 sequences)

SEQ ID NO: 1 - protein, 20 aa, synthetic construct
  REGION 1..20: note = signal peptide
MARPLCTLLLLMATLAGALA

SEQ ID NO: 2 - protein, 254 aa, synthetic construct
  REGION 1..254: note = 10E8v4-5R+100cF scFv
SELTQDPAVSVALKQTVTITCRGDSLRSHYASWYQKKPGQAPVLLFYGKNNRPSGIPDRFSGSASGNRASLTITGAQAEDEADYYCSSRDKSGSRLSVFGGGTKLTVLGGGGSGGGGSGGGGSEVRLRESGGGLVKPGGSLRLSCSASGFDFDNAWMTWVRQPPGKGLEWVGRITGPGEGWSVDYAESVKGRFTISRDNTKNTLYLEMNNVRTEDTGYYFCARTGKYYDFWFGYPPGEEYFQDWGQGTLVIVSS

SEQ ID NO: 3 - protein, 253 aa, synthetic construct
  REGION 1..253: note = Ibalizumab scFv
DIVMTQSPDSLAVSLGERVTMNCKSSQSLLYSTNQKNYLAWYQQKPGQSPKLLIYWASTRESGVPDRFSGSGSGTDFTLTISSVQAEDVAVYYCQQYYSYRTFGGGTKLEIKRTVAGGGGSGGGGSGGGGSQVQLQQSGPEVVKPGASVKMSCKASGYTFTSYVIHWVRQKPGQGLDWIGYINPYNDGTDYDEKFKGKATLTSDTSTSTAYMELSSLRSEDTAVYYCAREKDNYATGAWFAYWGQGTLVTVSS

SEQ ID NO: 4 - protein, 232 aa, synthetic construct
  REGION 1..232: note = Human IgG1 Fc fragment
EPKSCDKTHTCPPCPAPELLGGPSVFLFPPKPKDTLMISRTPEVTCVVVDVSHEDPEVKFNWYVDGVEVHNAKTKPREEQYNSTYRVVSVLTVLHQDWLNGKEYKCKVSNKALPAPIEKTISKAKGQPREPQVYTLPPSRDELTKNQVSLTCLVKGFYPSDIAVEWESNGQPENNYKTTPPVLDSDGSFFLYSKLTVDKSRWQQGNVFSCSVMHEALHNHYTQKSLSLSPGK

SEQ ID NO: 5 - protein, 28 aa, synthetic construct
  REGION 1..28: note = HIV membrane fusion-inhibiting peptide P52
WEQKIEELLKKAEEQQKKNEEELKKLEK

SEQ ID NO: 6 - protein, 36 aa, synthetic construct
  REGION 1..36: note = HIV membrane fusion-inhibiting peptide C34
YTSLIHSLIEESQNQQEKNEQELLELDKWASLWNWF

SEQ ID NO: 7 - protein, 34 aa, synthetic construct
  REGION 1..34: note = HIV membrane fusion-inhibiting peptide T20
LLEQENKEQQNQSEEILSHILSTYNNIERDWEMW

SEQ ID NO: 8 - protein, 784 aa, synthetic construct
  REGION 1..784: note = KL-BsHIV01
MARPLCTLLLLMATLAGALASELTQDPAVSVALKQTVTITCRGDSLRSHYASWYQKKPGQAPVLLFYGKNNRPSGIPDRFSGSASGNRASLTITGAQAEDEADYYCSSRDKSGSRLSVFGGGTKLTVLGGGGSGGGGSGGGGSEVRLRESGGGLVKPGGSLRLSCSASGFDFDNAWMTWVRQPPGKGLEWVGRITGPGEGWSVDYAESVKGRFTISRDNTKNTLYLEMNNVRTEDTGYYFCARTGKYYDFWFGYPPGEEYFQDWGQGTLVIVSSGGGGSGGGGSGGGGSGGGGSGGGGSDIVMTQSPDSLAVSLGERVTMNCKSSQSLLYSTNQKNYLAWYQQKPGQSPKLLIYWASTRESGVPDRFSGSGSGTDFTLTISSVQAEDVAVYYCQQYYSYRTFGGGTKLEIKRTVAGGGGSGGGGSGGGGSQVQLQQSGPEVVKPGASVKMSCKASGYTFTSYVIHWVRQKPGQGLDWIGYINPYNDGTDYDEKFKGKATLTSDTSTSTAYMELSSLRSEDTAVYYCAREKDNYATGAWFAYWGQGTLVTVSSEPKSCDKTHTCPPCPAPELLGGPSVFLFPPKPKDTLMISRTPEVTCVVVDVSHEDPEVKFNWYVDGVEVHNAKTKPREEQYNSTYRVVSVLTVLHQDWLNGKEYKCKVSNKALPAPIEKTISKAKGQPREPQVYTLPPSRDELTKNQVSLTCLVKGFYPSDIAVEWESNGQPENNYKTTPPVLDSDGSFFLYSKLTVDKSRWQQGNVFSCSVMHEALHNHYTQKSLSLSPGK

SEQ ID NO: 9 - DNA, 2355 bp, synthetic construct
  misc_feature 1..2355: note = KL-BsHIV01
  source 1..2355: mol_type = other DNA
atggcgagacccctgtgcacattacttctgttgatggctaccctggcaggcgccctcgccagcgagctgacacaggaccctgccgtgtccgtggccctgaagcagaccgtgacaatcacctgcagaggcgattccctgagatcccactacgcctcctggtaccagaagaagcctggccaggcccccgtgctgctgttttacggcaagaataaccgccccagcggcatccccgatagattttccggcagcgcctccggcaacagagccagcctgacaatcaccggcgcccaggccgaggacgaggctgattactactgcagctccagagataagagcggcagcagactgtccgtgtttggcggcggcaccaagctgaccgtgctcggaggaggaggaagcggaggaggaggctcaggcggcggcggctctgaggtgaggctgagagagtccggcggcggcctggtgaagcccggaggatctctgaggctgtcctgctccgcctccggcttcgattttgacaatgcctggatgacctgggtgagacagccccctggcaagggcctggagtgggtgggaaggatcacaggccccggcgagggctggtccgtggattacgccgagtccgtgaagggcaggttcacaatctccagggataacaccaagaacaccctgtacctggagatgaacaacgtgaggacagaggataccggctactacttttgcgccagaacaggcaagtactacgacttttggttcggctacccccctggcgaggagtacttccaggattggggccagggcaccctggtcattgtgtccagcggcggcggcggcagtggcggcggcggaagcggcggcggcggctctggcggcggcggcagcggcggcggcggctccgacatcgtgatgacccagtctcctgatagcctggccgtgagcctgggcgagagagtgacaatgaactgtaagtctagccagagcctgctgtactccaccaaccagaagaattacctggcctggtatcagcagaagcctggccagtccccaaagctgctgatctattgggcatctacaagggagagcggagtgccagacagattcagcggatccggatctggaaccgacttcaccctgacaatctcctctgtgcaggccgaggacgtggccgtgtactattgccagcagtactatagctacaggacattcggcggcggcaccaagctggagatcaagcgcaccgtggccggaggaggaggatctggcggaggagggtccggcggcggcggctcccaggtgcagctgcagcagagcggaccagaggtggtgaagcctggagcctccgtgaagatgtcttgtaaggccagcggctacaccttcacatcctatgtgatccactgggtgaggcagaagccaggacagggactggactggatcggctacatcaacccttataatgatggcaccgactacgatgagaagtttaagggcaaggccaccctgacatccgataccagcacatccaccgcctatatggagctgagctccctgcggtctgaggacacagccgtgtactattgcgccagagagaaggataactacgcaaccggagcatggttcgcatattggggacagggtaccctggtcaccgtgtctagcgagcccaagagctgtgacaagacacacacctgccctccatgtccagcaccagagctgctgggagggccctccgtgttcctgtttccccctaagccaaaggatacactgatgatctccaggacaccagaggtgacctgcgtggtggtggacgtgtctcacgaggatcctgaggtgaagtttaactggtacgtggacggcgtggaggtgcacaatgccaagaccaagcctagggaggagcagtacaattctacatatcgcgtggtgagcgtgctgaccgtgctgcaccaggattggctgaacggcaaggagtataagtgcaaggtgagcaataaggccctgcctgccccaatcgagaagacaatctccaaggcaaagggacagccaagggagcctcaggtgtacaccctgccaccctctcgcgacgagctgacaaagaaccaggtgagcctgacctgtctggtgaagggcttctatcctagcgatattgccgtggagtgggagtccaatggccagccagagaacaattacaagaccacacctccagtgctggactccgatggctctttctttctgtattccaagctgacagtggacaagtctagatggcagcagggcaacgtgttttcttgtagcgtgatgcacgaggccctgcacaatcactacacccagaagtccctgtctctgagccccggcaagtag

SEQ ID NO: 10 - protein, 837 aa, synthetic construct
  REGION 1..837: note = KL-BsHIV01-003
MARPLCTLLLLMATLAGALASELTQDPAVSVALKQTVTITCRGDSLRSHYASWYQKKPGQAPVLLFYGKNNRPSGIPDRFSGSASGNRASLTITGAQAEDEADYYCSSRDKSGSRLSVFGGGTKLTVLGGGGSGGGGSGGGGSEVRLRESGGGLVKPGGSLRLSCSASGFDFDNAWMTWVRQPPGKGLEWVGRITGPGEGWSVDYAESVKGRFTISRDNTKNTLYLEMNNVRTEDTGYYFCARTGKYYDFWFGYPPGEEYFQDWGQGTLVIVSSGGGGSGGGGSGGGGSGGGGSGGGGSDIVMTQSPDSLAVSLGERVTMNCKSSQSLLYSTNQKNYLAWYQQKPGQSPKLLIYWASTRESGVPDRFSGSGSGTDFTLTISSVQAEDVAVYYCQQYYSYRTFGGGTKLEIKRTVAGGGGSGGGGSGGGGSQVQLQQSGPEVVKPGASVKMSCKASGYTFTSYVIHWVRQKPGQGLDWIGYINPYNDGTDYDEKFKGKATLTSDTSTSTAYMELSSLRSEDTAVYYCAREKDNYATGAWFAYWGQGTLVTVSSEPKSCDKTHTCPPCPAPELLGGPSVFLFPPKPKDTLMISRTPEVTCVVVDVSHEDPEVKFNWYVDGVEVHNAKTKPREEQYNSTYRVVSVLTVLHQDWLNGKEYKCKVSNKALPAPIEKTISKAKGQPREPQVYTLPPSRDELTKNQVSLTCLVKGFYPSDIAVEWESNGQPENNYKTTPPVLDSDGSFFLYSKLTVDKSRWQQGNVFSCSVMHEALHNHYTQKSLSLSPGKGGGGSGGGGSGGGGSGGGGSGGGGSWEQKIEELLKKAEEQQKKNEEELKKLEK

SEQ ID NO: 11 - DNA, 2514 bp, synthetic construct
  misc_feature 1..2514: note = KL-BsHIV01-003
  source 1..2514: mol_type = other DNA
atggcgagacccctgtgcacattacttctgttgatggctaccctggcaggcgccctcgccagcgagctgacacaggaccctgccgtgtccgtggccctgaagcagaccgtgacaatcacctgcagaggcgattccctgagatcccactacgcctcctggtaccagaagaagcctggccaggcccccgtgctgctgttttacggcaagaataaccgccccagcggcatccccgatagattttccggcagcgcctccggcaacagagccagcctgacaatcaccggcgcccaggccgaggacgaggctgattactactgcagctccagagataagagcggcagcagactgtccgtgtttggcggcggcaccaagctgaccgtgctcggaggaggaggaagcggaggaggaggctcaggcggcggcggctctgaggtgaggctgagagagtccggcggcggcctggtgaagcccggaggatctctgaggctgtcctgctccgcctccggcttcgattttgacaatgcctggatgacctgggtgagacagccccctggcaagggcctggagtgggtgggaaggatcacaggccccggcgagggctggtccgtggattacgccgagtccgtgaagggcaggttcacaatctccagggataacaccaagaacaccctgtacctggagatgaacaacgtgaggacagaggataccggctactacttttgcgccagaacaggcaagtactacgacttttggttcggctacccccctggcgaggagtacttccaggattggggccagggcaccctggtcattgtgtccagcggcggcggcggcagtggcggcggcggaagcggcggcggcggctctggcggcggcggcagcggcggcggcggctccgacatcgtgatgacccagtctcctgatagcctggccgtgagcctgggcgagagagtgacaatgaactgtaagtctagccagagcctgctgtactccaccaaccagaagaattacctggcctggtatcagcagaagcctggccagtccccaaagctgctgatctattgggcatctacaagggagagcggagtgccagacagattcagcggatccggatctggaaccgacttcaccctgacaatctcctctgtgcaggccgaggacgtggccgtgtactattgccagcagtactatagctacaggacattcggcggcggcaccaagctggagatcaagcgcaccgtggccggaggaggaggatctggcggaggagggtccggcggcggcggctcccaggtgcagctgcagcagagcggaccagaggtggtgaagcctggagcctccgtgaagatgtcttgtaaggccagcggctacaccttcacatcctatgtgatccactgggtgaggcagaagccaggacagggactggactggatcggctacatcaacccttataatgatggcaccgactacgatgagaagtttaagggcaaggccaccctgacatccgataccagcacatccaccgcctatatggagctgagctccctgcggtctgaggacacagccgtgtactattgcgccagagagaaggataactacgcaaccggagcatggttcgcatattggggacagggtaccctggtcaccgtgtctagcgagcccaagagctgtgacaagacacacacctgccctccatgtccagcaccagagctgctgggagggccctccgtgttcctgtttccccctaagccaaaggatacactgatgatctccaggacaccagaggtgacctgcgtggtggtggacgtgtctcacgaggatcctgaggtgaagtttaactggtacgtggacggcgtggaggtgcacaatgccaagaccaagcctagggaggagcagtacaattctacatatcgcgtggtgagcgtgctgaccgtgctgcaccaggattggctgaacggcaaggagtataagtgcaaggtgagcaataaggccctgcctgccccaatcgagaagacaatctccaaggcaaagggacagccaagggagcctcaggtgtacaccctgccaccctctcgcgacgagctgacaaagaaccaggtgagcctgacctgtctggtgaagggcttctatcctagcgatattgccgtggagtgggagtccaatggccagccagagaacaattacaagaccacacctccagtgctggactccgatggctctttctttctgtattccaagctgacagtggacaagtctagatggcagcagggcaacgtgttttcttgtagcgtgatgcacgaggccctgcacaatcactacacccagaagtccctgtctctgagccccggcaagggcggaggaggaagcggaggaggcggctctggcggaggaggttccggaggaggcggaagcggcggaggaggctcttgggagcagaagatcgaggagctgctgaagaaggccgaggagcagcagaagaagaatgaggaggagctgaagaagctggagaagtag

SEQ ID NO: 12 - protein, 845 aa, synthetic construct
  REGION 1..845: note = KL-BsHIV01-C34
MARPLCTLLLLMATLAGALASELTQDPAVSVALKQTVTITCRGDSLRSHYASWYQKKPGQAPVLLFYGKNNRPSGIPDRFSGSASGNRASLTITGAQAEDEADYYCSSRDKSGSRLSVFGGGTKLTVLGGGGSGGGGSGGGGSEVRLRESGGGLVKPGGSLRLSCSASGFDFDNAWMTWVRQPPGKGLEWVGRITGPGEGWSVDYAESVKGRFTISRDNTKNTLYLEMNNVRTEDTGYYFCARTGKYYDFWFGYPPGEEYFQDWGQGTLVIVSSGGGGSGGGGSGGGGSGGGGSGGGGSDIVMTQSPDSLAVSLGERVTMNCKSSQSLLYSTNQKNYLAWYQQKPGQSPKLLIYWASTRESGVPDRFSGSGSGTDFTLTISSVQAEDVAVYYCQQYYSYRTFGGGTKLEIKRTVAGGGGSGGGGSGGGGSQVQLQQSGPEVVKPGASVKMSCKASGYTFTSYVIHWVRQKPGQGLDWIGYINPYNDGTDYDEKFKGKATLTSDTSTSTAYMELSSLRSEDTAVYYCAREKDNYATGAWFAYWGQGTLVTVSSEPKSCDKTHTCPPCPAPELLGGPSVFLFPPKPKDTLMISRTPEVTCVVVDVSHEDPEVKFNWYVDGVEVHNAKTKPREEQYNSTYRVVSVLTVLHQDWLNGKEYKCKVSNKALPAPIEKTISKAKGQPREPQVYTLPPSRDELTKNQVSLTCLVKGFYPSDIAVEWESNGQPENNYKTTPPVLDSDGSFFLYSKLTVDKSRWQQGNVFSCSVMHEALHNHYTQKSLSLSPGKGGGGSGGGGSGGGGSGGGGSGGGGSYTSLIHSLIEESQNQQEKNEQELLELDKWASLWNWF

SEQ ID NO: 13 - DNA, 2538 bp, synthetic construct
  misc_feature 1..2538: note = KL-BsHIV01-C34
  source 1..2538: mol_type = other DNA
atggcgagacccctgtgcacattacttctgttgatggctaccctggcaggcgccctcgcctccgagctgacccaggaccctgccgtcagcgtggccttgaaacagaccgtaactataacgtgcagaggtgatagcttaagatcccactacgccagctggtatcaaaagaagccaggtcaggctcccgtgctcctgttctacgggaagaataaccgcccatccggcattccggatcggttctccggaagcgcaagtggaaatcgcgcctcgctgacaataacaggagcgcaggcagaggacgaagcagactactattgttcaagtagggataagagcggatccaggctgagcgtgttcggcggaggcaccaagctgacagtgcttggtggggggggctccggcggcggcggcagcggaggagggggaagtgaggttagactgagggagtccggcggggggttagtcaagccagggggcagtctccggctttcctgctcagctagtggcttcgatttcgataacgcgtggatgacttgggtccgccagcctcccgggaaagggctcgagtgggtgggaagaatcacaggccccggcgagggatggtccgttgactatgcagagtctgtcaagggtcggttcactatcagccgagataataccaagaacactctgtacttggagatgaataacgtgagaacagaagacacaggatactacttctgtgctcgtactggcaaatattatgacttttggttcgggtacccaccgggagaggagtatttccaggactggggccagggtacactggtcattgtgtcttctggtggcggagggtctggcggaggcggatccggcggaggtggctcaggcggaggagggagtggcggcggcggttctgacatcgtaatgactcagtcaccagactctctggccgtatccttaggagagcgcgtgacgatgaactgcaagtcttctcagtcactgctttacagcacaaaccaaaaaaactacctggcttggtaccagcagaagcctggacagagccccaagctactgatctattgggcctcgactagagaaagtggggtgcccgacagattttcggggagtggcagcggtacagattttacactcaccatttcctcagtgcaggcagaagatgtggccgtgtactattgccaacagtattacagctatcggacatttggtggtggcacaaagctagagattaagaggaccgtggccggaggtggcggcagtggagggggcgggagtgggggcggaggttcacaggtgcagctgcaacagtccgggcctgaagtggttaaacccggagcgagcgtaaagatgtcttgcaaggcttccggttatacattcacatcatatgtcattcactgggtgaggcaaaagccagggcaaggtcttgattggatagggtacatcaatccttacaatgatgggactgactacgatgagaagttcaagggaaaggcaaccctgacttctgatacctccacgtctaccgcttacatggaactaagctccctgcgttcagaggacactgccgtgtactattgtgctcgggagaaagataactatgccaccggcgcctggtttgcctactggggccaaggcaccttggtgaccgttagctccgagccgaaatcgtgcgacaagacccacacctgtcccccctgtcctgcacctgagctcctgggtgggccctctgtattcctcttccctccaaaaccaaaagacacgttgatgattagcaggaccccagaagtaacatgcgttgtggtcgacgtctcacatgaagacccagaggtgaaatttaattggtacgtcgatggggttgaagttcataacgccaaaactaagccgagggaggaacagtataatagcacttatcgagtggtttcagttttgaccgtacttcatcaagactggctgaacgggaaggaatataagtgcaaggtgagtaataaagcactgcctgcgcccatcgagaaaacgatcagtaaagccaagggacagcctcgcgaaccccaggtgtacactcttccgccctcccgggacgagctcaccaaaaaccaggtgtccttgacctgtctcgtcaagggcttttacccatcagatatcgctgtcgaatgggaaagtaacgggcagcctgaaaacaattacaaaacaaccccacccgtcctcgattcagatggcagcttttttttatactctaaacttacggtggacaaatctcgctggcaacaggggaatgtgtttagctgcagcgtcatgcacgaagctctgcataaccactatacccagaaaagcctgtctctcagccccgggaaaggcggaggaggaagcggaggaggcggctctggcggaggaggttccggaggaggcggaagcggcggaggaggctcttacacctccctgatccactccctgatcgaggagtcccagaatcagcaggagaagaatgagcaggagctgctggagctggataagtgggcctccctgtggaattggttctag

SEQ ID NO: 14 - protein, 843 aa, synthetic construct
  REGION 1..843: note = KL-BsHIV01-T20
MARPLCTLLLLMATLAGALASELTQDPAVSVALKQTVTITCRGDSLRSHYASWYQKKPGQAPVLLFYGKNNRPSGIPDRFSGSASGNRASLTITGAQAEDEADYYCSSRDKSGSRLSVFGGGTKLTVLGGGGSGGGGSGGGGSEVRLRESGGGLVKPGGSLRLSCSASGFDFDNAWMTWVRQPPGKGLEWVGRITGPGEGWSVDYAESVKGRFTISRDNTKNTLYLEMNNVRTEDTGYYFCARTGKYYDFWFGYPPGEEYFQDWGQGTLVIVSSGGGGSGGGGSGGGGSGGGGSGGGGSDIVMTQSPDSLAVSLGERVTMNCKSSQSLLYSTNQKNYLAWYQQKPGQSPKLLIYWASTRESGVPDRFSGSGSGTDFTLTISSVQAEDVAVYYCQQYYSYRTFGGGTKLEIKRTVAGGGGSGGGGSGGGGSQVQLQQSGPEVVKPGASVKMSCKASGYTFTSYVIHWVRQKPGQGLDWIGYINPYNDGTDYDEKFKGKATLTSDTSTSTAYMELSSLRSEDTAVYYCAREKDNYATGAWFAYWGQGTLVTVSSEPKSCDKTHTCPPCPAPELLGGPSVFLFPPKPKDTLMISRTPEVTCVVVDVSHEDPEVKFNWYVDGVEVHNAKTKPREEQYNSTYRVVSVLTVLHQDWLNGKEYKCKVSNKALPAPIEKTISKAKGQPREPQVYTLPPSRDELTKNQVSLTCLVKGFYPSDIAVEWESNGQPENNYKTTPPVLDSDGSFFLYSKLTVDKSRWQQGNVFSCSVMHEALHNHYTQKSLSLSPGKGGGGSGGGGSGGGGSGGGGSGGGGSLLEQENKEQQNQSEEILSHILSTYNNIERDWEMW

SEQ ID NO: 15 - protein, 2532 aa, synthetic construct
  REGION 1..2532: note = KL-BsHIV01-T20
ATGGCGAGACCCCTGTGCACATTACTTCTGTTGATGGCTACCCTGGCAGGCGCCCTCGCCAGCGAGCTGACACAGGACCCTGCCGTGTCCGTGGCCCTGAAGCAGACCGTGACAATCACCTGCAGAGGCGATTCCCTGAGATCCCACTACGCCTCCTGGTACCAGAAGAAGCCTGGCCAGGCCCCCGTGCTGCTGTTTTACGGCAAGAATAACCGCCCCAGCGGCATCCCCGATAGATTTTCCGGCAGCGCCTCCGGCAACAGAGCCAGCCTGACAATCACCGGCGCCCAGGCCGAGGACGAGGCTGATTACTACTGCAGCTCCAGAGATAAGAGCGGCAGCAGACTGTCCGTGTTTGGCGGCGGCACCAAGCTGACCGTGCTCGGAGGAGGAGGAAGCGGAGGAGGAGGCTCAGGCGGCGGCGGCTCTGAGGTGAGGCTGAGAGAGTCCGGCGGCGGCCTGGTGAAGCCCGGAGGATCTCTGAGGCTGTCCTGCTCCGCCTCCGGCTTCGATTTTGACAATGCCTGGATGACCTGGGTGAGACAGCCCCCTGGCAAGGGCCTGGAGTGGGTGGGAAGGATCACAGGCCCCGGCGAGGGCTGGTCCGTGGATTACGCCGAGTCCGTGAAGGGCAGGTTCACAATCTCCAGGGATAACACCAAGAACACCCTGTACCTGGAGATGAACAACGTGAGGACAGAGGATACCGGCTACTACTTTTGCGCCAGAACAGGCAAGTACTACGACTTTTGGTTCGGCTACCCCCCTGGCGAGGAGTACTTCCAGGATTGGGGCCAGGGCACCCTGGTCATTGTGTCCAGCGGCGGCGGCGGCAGTGGCGGCGGCGGAAGCGGCGGCGGCGGCTCTGGCGGCGGCGGCAGCGGCGGCGGCGGCTCCGACATCGTGATGACCCAGTCTCCTGATAGCCTGGCCGTGAGCCTGGGCGAGAGAGTGACAATGAACTGTAAGTCTAGCCAGAGCCTGCTGTACTCCACCAACCAGAAGAATTACCTGGCCTGGTATCAGCAGAAGCCTGGCCAGTCCCCAAAGCTGCTGATCTATTGGGCATCTACAAGGGAGAGCGGAGTGCCAGACAGATTCAGCGGATCCGGATCTGGAACCGACTTCACCCTGACAATCTCCTCTGTGCAGGCCGAGGACGTGGCCGTGTACTATTGCCAGCAGTACTATAGCTACAGGACATTCGGCGGCGGCACCAAGCTGGAGATCAAGCGCACCGTGGCCGGAGGAGGAGGATCTGGCGGAGGAGGGTCCGGCGGCGGCGGCTCCCAGGTGCAGCTGCAGCAGAGCGGACCAGAGGTGGTGAAGCCTGGAGCCTCCGTGAAGATGTCTTGTAAGGCCAGCGGCTACACCTTCACATCCTATGTGATCCACTGGGTGAGGCAGAAGCCAGGACAGGGACTGGACTGGATCGGCTACATCAACCCTTATAATGATGGCACCGACTACGATGAGAAGTTTAAGGGCAAGGCCACCCTGACATCCGATACCAGCACATCCACCGCCTATATGGAGCTGAGCTCCCTGCGGTCTGAGGACACAGCCGTGTACTATTGCGCCAGAGAGAAGGATAACTACGCAACCGGAGCATGGTTCGCATATTGGGGACAGGGTACCCTGGTCACCGTGTCTAGCGAGCCCAAGAGCTGTGACAAGACACACACCTGCCCTCCATGTCCAGCACCAGAGCTGCTGGGAGGGCCCTCCGTGTTCCTGTTTCCCCCTAAGCCAAAGGATACACTGATGATCTCCAGGACACCAGAGGTGACCTGCGTGGTGGTGGACGTGTCTCACGAGGATCCTGAGGTGAAGTTTAACTGGTACGTGGACGGCGTGGAGGTGCACAATGCCAAGACCAAGCCTAGGGAGGAGCAGTACAATTCTACATATCGCGTGGTGAGCGTGCTGACCGTGCTGCACCAGGATTGGCTGAACGGCAAGGAGTATAAGTGCAAGGTGAGCAATAAGGCCCTGCCTGCCCCAATCGAGAAGACAATCTCCAAGGCAAAGGGACAGCCAAGGGAGCCTCAGGTGTACACCCTGCCACCCTCTCGCGACGAGCTGACAAAGAACCAGGTGAGCCTGACCTGTCTGGTGAAGGGCTTCTATCCTAGCGATATTGCCGTGGAGTGGGAGTCCAATGGCCAGCCAGAGAACAATTACAAGACCACACCTCCAGTGCTGGACTCCGATGGCTCTTTCTTTCTGTATTCCAAGCTGACAGTGGACAAGTCTAGATGGCAGCAGGGCAACGTGTTTTCTTGTAGCGTGATGCACGAGGCCCTGCACAATCACTACACCCAGAAGTCCCTGTCTCTGAGCCCCGGCAAGGGCGGAGGAGGAAGCGGAGGAGGCGGCTCTGGCGGAGGAGGTTCCGGAGGAGGCGGAAGCGGCGGAGGAGGCTCTCTGCTGGAGCAGGAGAACAAGGAGCAGCAGAATCAGAGCGAGGAGATCCTGTCCCACATCCTGTCCACATACAACAATATCGAGAGAGATTGGGAGATGTGGTAG

SEQ ID NO: 16 - DNA, 7128 bp, synthetic construct
  misc_feature 1..7128: note = pKL-kan-lenti-EF1-WPRE
  source 1..7128: mol_type = other DNA
ggccgcgttgctggcgtttttccataggctccgcccccctgacgagcatcacaaaaatcgacgctcaagtcagaggtggcgaaacccgacaggactataaagataccaggcgtttccccctggaagctccctcgtgcgctctcctgttccgaccctgccgcttaccggatacctgtccgcctttctcccttcgggaagcgtggcgctttctcatagctcacgctgtaggtatctcagttcggtgtaggtcgttcgctccaagctgggctgtgtgcacgaaccccccgttcagcccgaccgctgcgccttatccggtaactatcgtcttgagtccaacccggtaagacacgacttatcgccactggcagcagccactggtaacaggattagcagagcgaggtatgtaggcggtgctacagagttcttgaagtggtggcctaactacggctacactagaagaacagtatttggtatctgcgctctgctgaagccagttaccttcggaaaaagagttggtagctcttgatccggcaaacaaaccaccgctggtagcggtggtttttttgtttgcaagcagcagattacgcgcagaaaaaaaggatctcaagaagatcctttgatcttttctacggggtctgacgctcagtggaacgaaaactcacgttaagggattttggtcatgaagcgcttttgaagctcggatccgaacaaacgacccaacacccgtgcgttttattctgtctttttattgccgatcccctcagaagaactcgtcaagaaggcgatagaaggcgatgcgctgcgaatcgggagcggcgataccgtaaagcacgaggaagcggtcagcccattcgccgccaagctcttcagcaatatcacgggtagccaacgctatgtcctgatagcggtccgccacacccagccggccacagtcgatgaatccagaaaagcggccattttccaccatgatattcggcaagcaggcatcgccatgggtcacgacgagatcctcgccgtcgggcatgctcgccttgagcctggcgaacagttcggctggcgcgagcccctgatgctcttcgtccagatcatcctgatcgacaagaccggcttccatccgagtacgtgctcgctcgatgcgatgtttcgcttggtggtcgaatgggcaggtagccggatcaagcgtatgcagccgccgcattgcatcagccatgatggatactttctcggcaggagcaaggtgagatgacaggagatcctgccccggcacttcgcccaatagcagccagtcccttcccgcttcagtgacaacgtcgagcacagctgcgcaaggaacgcccgtcgtggccagccacgatagccgcgctgcctcgtcttgcagttcattcagggcaccggacaggtcggtcttgacaaaaagaaccgggcgcccctgcgctgacagccggaacacggcggcatcagagcagccgattgtctgttgtgcccagtcatagccgaatagcctctccacccaagcggccggagaacctgcgtgcaatccatcttgttcaatcatgcgaaacgatcctcatcctgtctcttgatcagagcttgatcccctgcgccatcagatccttggcggcaagaaagccatccagtttactttgcagggcttcccaaccttaccagaggcctgcgccgcggccagctggctagcaattcccgggttaactctagagacattgattattgactagttattaatagtaatcaattacggggtcattagttcatagcccatatatggagttccgcgttacataacttacggtaaatggcccgcctggctgaccgcccaacgacccccgcccattgacgtcaataatgacgtatgttcccatagtaacgccaatagggactttccattgacgtcaatgggtggagtatttacggtaaactgcccacttggcagtacatcaagtgtatcatatgccaagtacgccccctattgacgtcaatgacggtaaatggcccgcctggcattatgcccagtacatgaccttatgggactttcctacttggcagtacatctacgtattagtcatcgctattaccatggtgatgcggttttggcagtacatcaatgggcgtggatagcggtttgactcacggggatttccaagtctccaccccattgacgtcaatgggagtttgttttggcaccaaaatcaacgggactttccaaaatgtcgtaacaactccgccccattgacgcaaatgggcggtaggcgtgtacggtgggaggtctatataagcagagctcgtttagtgaaccggggtctctctggttagaccagatctgagcctgggagctctctggctaactagggaacccactgcttaagcctcaataaagcttgccttgagtgcttcaagtagtgtgtgcccgtctgttgtgtgactctggtaactagagatccctcagacccttttagtcagtgtggaaaatctctagcagtggcgcccgaacagggacttgaaagcgaaagggaaaccagaggagctctctcgacgcaggactcggcttgctgaagcgcgcacggcaagaggcgaggggcggcgactggtgagtacgccaaaaattttgactagcggaggctagaaggagagagatgggtgcgagagcgtcagtattaagcgggggagaattagatcgcgatgggaaaaaattcggttaaggccagggggaaagaaaaaatataaattaaaacatatagtatgggcaagcagggagctagaacgattcgcagttaatcctggcctgttagaaacatcagaaggctgtagacaaatactgggacagctacaaccatcccttcagacaggatcagaagaacttagatcattatataatacagtagcaaccctctattgtgtgcatcaaaggatagagataaaagacaccaaggaagctttagacaagatagaggaagagcaaaacaaaagtaagaccaccgcacagcaagcggccgctgatcttcagacctggaggaggagatatgagggacaattggagaagtgaattatataaatataaagtagtaaaaattgaaccattaggagtagcacccaccaaggcaaagagaagagtggtgcagagagaaaaaagagcagtgggaataggagctttgttccttgggttcttgggagcagcaggaagcactatgggcgcagcgtcaatgacgctgacggtacaggccagacaattattgtctggtatagtgcagcagcagaacaatttgctgagggctattgaggcgcaacagcatctgttgcaactcacagtctggggcatcaagcagctccaggcaagaatcctggctgtggaaagatacctaaaggatcaacagctcctggggatttggggttgctctggaaaactcatttgcaccactgctgtgccttggaatgctagttggagtaataaatctctggaacagatttggaatcacacgacctggatggagtgggacagagaaattaacaattacacaagcttaatacactccttaattgaagaatcgcaaaaccagcaagaaaagaatgaacaagaattattggaattagataaatgggcaagtttgtggaattggtttaacataacaaattggctgtggtatataaaattattcataatgatagtaggaggcttggtaggtttaagaatagtttttgctgtactttctatagtgaatagagttaggcagggatattcaccattatcgtttcagacccacctcccaaccccgaggggacccgacaggcccgaaggaatagaagaagaaggtggagagagagacagagacagatccattcgattagtgaacggatctcgacggtatcggttaacttttaaaagaaaaggggggattggggggtacagtgcaggggaaagaatagtagacataatagcaacagacatacaaactaaagaattacaaaaacaaattacaaaaattcaaaattttatcgatcacgagactagcctcgaggcatgcctgcaggaattcgctccggtgcccgtcagtgggcagagcgcacatcgcccacagtccccgagaagttggggggaggggtcggcaattgaaccggtgcctagagaaggtggcgcggggtaaactgggaaagtgatgtcgtgtactggctccgcctttttcccgagggtgggggagaaccgtatataagtgcagtagtcgccgtgaacgttctttttcgcaacgggtttgccgccagaacacaggtaagtgccgtgtgtggttcccgcgggcctggcctctttacgggttatggcccttgcgtgccttgaattacttccacgcccctggctgcagtacgtgattcttgatcccgagcttcgggttggaagtgggtgggagagttcgaggccttgcgcttaaggagccccttcgcctcgtgcttgagttgaggcctggcttgggcgctggggccgccgcgtgcgaatctggtggcaccttcgcgcctgtctcgctgctttcgataagtctctagccatttaaaatttttgatgacctgctgcgacgctttttttctggcaagatagtcttgtaaatgcgggccaagatctgcacactggtatttcggtttttggggccgcgggcggcgacggggcccgtgcgtcccagcgcacatgttcggcgaggcggggcctgcgagcgcggccaccgagaatcggacgggggtagtctcaagctggccggcctgctctggtgcctggcctcgcgccgccgtgtatcgccccgccctgggcggcaaggctggcccggtcggcaccagttgcgtgagcggaaagatggccgcttcccggccctgctgcagggagctcaaaatggaggacgcggcgctcgggagagcgggcgggtgagtcacccacacaaaggaaaagggcctttccgtcctcagccgtcgcttcatgtgactccacggagtaccgggcgccgtccaggcacctcgattagttctcgagcttttggagtacgtcgtctttaggttggggggaggggttttatgcgatggagtttccccacactgagtgggtggagactgaagttaggccagcttggcacttgatgtaattctccttggaatttgccctttttgagtttggatcttggttcattctcaagcctcagacagtggttcaaagtttttttcttccatttcaggtgtcgtgaggatctatttccggtgagacccaagctggctagctaaacttacgcgtgcctcggatcctccagtgtggtgtgcagatatccagcacagtcccgggccgagtctagacgtttaaacccgctgatcaggtcgacaatcaacctctggattacaaaatttgtgaaagattgactggtattcttaactatgttgctccttttacgctatgtggatacgctgctttaatgcctttgtatcatgctattgcttcccgtatggctttcattttctcctccttgtataaatcctggttgctgtctctttatgaggagttgtggcccgttgtcaggcaacgtggcgtggtgtgcactgtgtttgctgacgcaacccccactggttggggcattgccaccacctgtcagctcctttccgggactttcgctttccccctccctattgccacggcggaactcatcgccgcctgccttgcccgctgctggacaggggctcggctgttgggcactgacaattccgtggtgttgtcggggaagctgacgtcctttccatggctgctcgcctgtgttgccacctggattctgcgcgggacgtccttctgctacgtcccttcggccctcaatccagcggaccttccttcccgcggcctgctgccggctctgcggcctcttccgcgtcttcgccttcgccctcagacgagtcggatctccctttgggccgcctccccgcggtacctttaagaccaatgacttacaaggcagctgtagatcttagccactttttaaaagaaaaggggggactggaagggctaattcactcccaacgaagacaagatctgctttttgcttgtactgggtctctctggttagaccagatctgagcctgggagctctctggctaactagggaacccactgcttaagcctcaataaagcttgccttgagtgcttcaagtagtgtgtgcccgtctgttgtgtgactctggtaactagagatccctcagacccttttagtcagtgtggaaaatctctagcagtagtagttcatgtcatcttattattcagtatttataacttgcaaagaaatgaatatcagagagtgagaggaacttgtttattgcagcttataatggttacaaataaagcaatagcatcacaaatttcacaaataaagcatttttttcactgcattctagttgtggtttgtccaaactcatcaatgtatcttatcatgtctggctctagctatcccgcccctaactccgcccatcccgcccctaactccgcccagttccgcccattctccgccccatggctgactaattttttttatttatgcagaggccgaggccgcctcggcctctgagctattccagaagtagtgaggaggcttttttggaggccgctagcgtcgaccattacttattgttttagctgtcctcatgaatgtcttttcactacccatttgcttatcctgcatctctcagccttgactccactcagttctcttgcttagagataccacctttcccctgaagtgttccttccatgttttacggcgagatggtttctcctcgcctggccactcagccttagttgtctctgttgtcttatagaggtctacttgaagaaggaaaaacagggggcatggtttgactgtcctgtgagcccttcttccctgcctcccccactcacagtgacccggaatccctcgacatggcagtctagcactagtgcggccgcagatctgcttcctcgctcactgactcgctgcgctcggtcgttcggctgcggcgagcggtatcagctcactcaaaggcggtaatacggttatccacagaatcaggggataacgcaggaaagaacatgtgagcaaaaggccagcaaaaggccaggaaccgtaaaaa

SEQ ID NO: 17 - DNA, 814 bp, synthetic construct
  misc_feature 1..814: note = CBH promoter
  source 1..814: mol_type = other DNA
cgttacataacttacggtaaatggcccgcctggctgaccgcccaacgacccccgcccattgacgtcaataatgacgtatgttcccatagtaacgccaatagggactttccattgacgtcaatgggtggagtatttacggtaaactgcccacttggcagtacatcaagtgtatcatatgccaagtacgccccctattgacgtcaatgacggtaaatggcccgcctggcattatgcccagtacatgaccttatgggactttcctacttggcagtacatctacgtattagtcatcgctattaccatggtcgaggtgagccccacgttctgcttcactctccccatctcccccccctccccacccccaattttgtatttatttattttttaattattttgtgcagcgatgggggcggggggggggggggggcgcgcgccaggcggggcggggcggggcgaggggcggggcggggcgaggcggagaggtgcggcggcagccaatcagagcggcgcgctccgaaagtttccttttatggcgaggcggcggcggcggcggccctataaaaagcgaagcgcgcggcgggcgggagtcgctgcgacgctgccttcgccccgtgccccgctccgccgccgcctcgcgccgcccgccccggctctgactgaccgcgttactcccacaggtgagcgggcgggacggcccttctcctccgggctgtaattagctgagcaagaggtaagggtttaagggatggttggttggtggggtattaatgtttaattacctggagcacctgcctgaaatcactttttttcaggt

SEQ ID NO: 18 - DNA, 9054 bp, synthetic construct
  misc_feature 1..9054: note = pKL-Kan-lenti-CBH-KL-BsHIV01
  source 1..9054: mol_type = other DNA
ggccgcgttgctggcgtttttccataggctccgcccccctgacgagcatcacaaaaatcgacgctcaagtcagaggtggcgaaacccgacaggactataaagataccaggcgtttccccctggaagctccctcgtgcgctctcctgttccgaccctgccgcttaccggatacctgtccgcctttctcccttcgggaagcgtggcgctttctcatagctcacgctgtaggtatctcagttcggtgtaggtcgttcgctccaagctgggctgtgtgcacgaaccccccgttcagcccgaccgctgcgccttatccggtaactatcgtcttgagtccaacccggtaagacacgacttatcgccactggcagcagccactggtaacaggattagcagagcgaggtatgtaggcggtgctacagagttcttgaagtggtggcctaactacggctacactagaagaacagtatttggtatctgcgctctgctgaagccagttaccttcggaaaaagagttggtagctcttgatccggcaaacaaaccaccgctggtagcggtggtttttttgtttgcaagcagcagattacgcgcagaaaaaaaggatctcaagaagatcctttgatcttttctacggggtctgacgctcagtggaacgaaaactcacgttaagggattttggtcatgaagcgcttttgaagctcggatccgaacaaacgacccaacacccgtgcgttttattctgtctttttattgccgatcccctcagaagaactcgtcaagaaggcgatagaaggcgatgcgctgcgaatcgggagcggcgataccgtaaagcacgaggaagcggtcagcccattcgccgccaagctcttcagcaatatcacgggtagccaacgctatgtcctgatagcggtccgccacacccagccggccacagtcgatgaatccagaaaagcggccattttccaccatgatattcggcaagcaggcatcgccatgggtcacgacgagatcctcgccgtcgggcatgctcgccttgagcctggcgaacagttcggctggcgcgagcccctgatgctcttcgtccagatcatcctgatcgacaagaccggcttccatccgagtacgtgctcgctcgatgcgatgtttcgcttggtggtcgaatgggcaggtagccggatcaagcgtatgcagccgccgcattgcatcagccatgatggatactttctcggcaggagcaaggtgagatgacaggagatcctgccccggcacttcgcccaatagcagccagtcccttcccgcttcagtgacaacgtcgagcacagctgcgcaaggaacgcccgtcgtggccagccacgatagccgcgctgcctcgtcttgcagttcattcagggcaccggacaggtcggtcttgacaaaaagaaccgggcgcccctgcgctgacagccggaacacggcggcatcagagcagccgattgtctgttgtgcccagtcatagccgaatagcctctccacccaagcggccggagaacctgcgtgcaatccatcttgttcaatcatgcgaaacgatcctcatcctgtctcttgatcagagcttgatcccctgcgccatcagatccttggcggcaagaaagccatccagtttactttgcagggcttcccaaccttaccagaggcctgcgccgcggccagctggctagcaattcccgggttaactctagagacattgattattgactagttattaatagtaatcaattacggggtcattagttcatagcccatatatggagttccgcgttacataacttacggtaaatggcccgcctggctgaccgcccaacgacccccgcccattgacgtcaataatgacgtatgttcccatagtaacgccaatagggactttccattgacgtcaatgggtggagtatttacggtaaactgcccacttggcagtacatcaagtgtatcatatgccaagtacgccccctattgacgtcaatgacggtaaatggcccgcctggcattatgcccagtacatgaccttatgggactttcctacttggcagtacatctacgtattagtcatcgctattaccatggtgatgcggttttggcagtacatcaatgggcgtggatagcggtttgactcacggggatttccaagtctccaccccattgacgtcaatgggagtttgttttggcaccaaaatcaacgggactttccaaaatgtcgtaacaactccgccccattgacgcaaatgggcggtaggcgtgtacggtgggaggtctatataagcagagctcgtttagtgaaccggggtctctctggttagaccagatctgagcctgggagctctctggctaactagggaacccactgcttaagcctcaataaagcttgccttgagtgcttcaagtagtgtgtgcccgtctgttgtgtgactctggtaactagagatccctcagacccttttagtcagtgtggaaaatctctagcagtggcgcccgaacagggacttgaaagcgaaagggaaaccagaggagctctctcgacgcaggactcggcttgctgaagcgcgcacggcaagaggcgaggggcggcgactggtgagtacgccaaaaattttgactagcggaggctagaaggagagagatgggtgcgagagcgtcagtattaagcgggggagaattagatcgcgatgggaaaaaattcggttaaggccagggggaaagaaaaaatataaattaaaacatatagtatgggcaagcagggagctagaacgattcgcagttaatcctggcctgttagaaacatcagaaggctgtagacaaatactgggacagctacaaccatcccttcagacaggatcagaagaacttagatcattatataatacagtagcaaccctctattgtgtgcatcaaaggatagagataaaagacaccaaggaagctttagacaagatagaggaagagcaaaacaaaagtaagaccaccgcacagcaagcggccgctgatcttcagacctggaggaggagatatgagggacaattggagaagtgaattatataaatataaagtagtaaaaattgaaccattaggagtagcacccaccaaggcaaagagaagagtggtgcagagagaaaaaagagcagtgggaataggagctttgttccttgggttcttgggagcagcaggaagcactatgggcgcagcgtcaatgacgctgacggtacaggccagacaattattgtctggtatagtgcagcagcagaacaatttgctgagggctattgaggcgcaacagcatctgttgcaactcacagtctggggcatcaagcagctccaggcaagaatcctggctgtggaaagatacctaaaggatcaacagctcctggggatttggggttgctctggaaaactcatttgcaccactgctgtgccttggaatgctagttggagtaataaatctctggaacagatttggaatcacacgacctggatggagtgggacagagaaattaacaattacacaagcttaatacactccttaattgaagaatcgcaaaaccagcaagaaaagaatgaacaagaattattggaattagataaatgggcaagtttgtggaattggtttaacataacaaattggctgtggtatataaaattattcataatgatagtaggaggcttggtaggtttaagaatagtttttgctgtactttctatagtgaatagagttaggcagggatattcaccattatcgtttcagacccacctcccaaccccgaggggacccgacaggcccgaaggaatagaagaagaaggtggagagagagacagagacagatccattcgattagtgaacggatctcgacggtatcggttaacttttaaaagaaaaggggggattggggggtacagtgcaggggaaagaatagtagacataatagcaacagacatacaaactaaagaattacaaaaacaaattacaaaaattcaaaattttatcgatcacgagactagcctcgaggcatgcctgcaggaattccgttacataacttacggtaaatggcccgcctggctgaccgcccaacgacccccgcccattgacgtcaataatgacgtatgttcccatagtaacgccaatagggactttccattgacgtcaatgggtggagtatttacggtaaactgcccacttggcagtacatcaagtgtatcatatgccaagtacgccccctattgacgtcaatgacggtaaatggcccgcctggcattatgcccagtacatgaccttatgggactttcctacttggcagtacatctacgtattagtcatcgctattaccatggtcgaggtgagccccacgttctgcttcactctccccatctcccccccctccccacccccaattttgtatttatttattttttaattattttgtgcagcgatgggggcggggggggggggggggcgcgcgccaggcggggcggggcggggcgaggggcggggcggggcgaggcggagaggtgcggcggcagccaatcagagcggcgcgctccgaaagtttccttttatggcgaggcggcggcggcggcggccctataaaaagcgaagcgcgcggcgggcgggagtcgctgcgacgctgccttcgccccgtgccccgctccgccgccgcctcgcgccgcccgccccggctctgactgaccgcgttactcccacaggtgagcgggcgggacggcccttctcctccgggctgtaattagctgagcaagaggtaagggtttaagggatggttggttggtggggtattaatgtttaattacctggagcacctgcctgaaatcactttttttcaggtaccggtcgccaccatggcgagacccctgtgcacattacttctgttgatggctaccctggcaggcgccctcgccagcgagctgacacaggaccctgccgtgtccgtggccctgaagcagaccgtgacaatcacctgcagaggcgattccctgagatcccactacgcctcctggtaccagaagaagcctggccaggcccccgtgctgctgttttacggcaagaataaccgccccagcggcatccccgatagattttccggcagcgcctccggcaacagagccagcctgacaatcaccggcgcccaggccgaggacgaggctgattactactgcagctccagagataagagcggcagcagactgtccgtgtttggcggcggcaccaagctgaccgtgctcggaggaggaggaagcggaggaggaggctcaggcggcggcggctctgaggtgaggctgagagagtccggcggcggcctggtgaagcccggaggatctctgaggctgtcctgctccgcctccggcttcgattttgacaatgcctggatgacctgggtgagacagccccctggcaagggcctggagtgggtgggaaggatcacaggccccggcgagggctggtccgtggattacgccgagtccgtgaagggcaggttcacaatctccagggataacaccaagaacaccctgtacctggagatgaacaacgtgaggacagaggataccggctactacttttgcgccagaacaggcaagtactacgacttttggttcggctacccccctggcgaggagtacttccaggattggggccagggcaccctggtcattgtgtccagcggcggcggcggcagtggcggcggcggaagcggcggcggcggctctggcggcggcggcagcggcggcggcggctccgacatcgtgatgacccagtctcctgatagcctggccgtgagcctgggcgagagagtgacaatgaactgtaagtctagccagagcctgctgtactccaccaaccagaagaattacctggcctggtatcagcagaagcctggccagtccccaaagctgctgatctattgggcatctacaagggagagcggagtgccagacagattcagcggatccggatctggaaccgacttcaccctgacaatctcctctgtgcaggccgaggacgtggccgtgtactattgccagcagtactatagctacaggacattcggcggcggcaccaagctggagatcaagcgcaccgtggccggaggaggaggatctggcggaggagggtccggcggcggcggctcccaggtgcagctgcagcagagcggaccagaggtggtgaagcctggagcctccgtgaagatgtcttgtaaggccagcggctacaccttcacatcctatgtgatccactgggtgaggcagaagccaggacagggactggactggatcggctacatcaacccttataatgatggcaccgactacgatgagaagtttaagggcaaggccaccctgacatccgataccagcacatccaccgcctatatggagctgagctccctgcggtctgaggacacagccgtgtactattgcgccagagagaaggataactacgcaaccggagcatggttcgcatattggggacagggtaccctggtcaccgtgtctagcgagcccaagagctgtgacaagacacacacctgccctccatgtccagcaccagagctgctgggagggccctccgtgttcctgtttccccctaagccaaaggatacactgatgatctccaggacaccagaggtgacctgcgtggtggtggacgtgtctcacgaggatcctgaggtgaagtttaactggtacgtggacggcgtggaggtgcacaatgccaagaccaagcctagggaggagcagtacaattctacatatcgcgtggtgagcgtgctgaccgtgctgcaccaggattggctgaacggcaaggagtataagtgcaaggtgagcaataaggccctgcctgccccaatcgagaagacaatctccaaggcaaagggacagccaagggagcctcaggtgtacaccctgccaccctctcgcgacgagctgacaaagaaccaggtgagcctgacctgtctggtgaagggcttctatcctagcgatattgccgtggagtgggagtccaatggccagccagagaacaattacaagaccacacctccagtgctggactccgatggctctttctttctgtattccaagctgacagtggacaagtctagatggcagcagggcaacgtgttttcttgtagcgtgatgcacgaggccctgcacaatcactacacccagaagtccctgtctctgagccccggcaagtaggatatccagcacagtcccgggccgagtctagacgtttaaacccgctgatcaggtcgacaatcaacctctggattacaaaatttgtgaaagattgactggtattcttaactatgttgctccttttacgctatgtggatacgctgctttaatgcctttgtatcatgctattgcttcccgtatggctttcattttctcctccttgtataaatcctggttgctgtctctttatgaggagttgtggcccgttgtcaggcaacgtggcgtggtgtgcactgtgtttgctgacgcaacccccactggttggggcattgccaccacctgtcagctcctttccgggactttcgctttccccctccctattgccacggcggaactcatcgccgcctgccttgcccgctgctggacaggggctcggctgttgggcactgacaattccgtggtgttgtcggggaagctgacgtcctttccatggctgctcgcctgtgttgccacctggattctgcgcgggacgtccttctgctacgtcccttcggccctcaatccagcggaccttccttcccgcggcctgctgccggctctgcggcctcttccgcgtcttcgccttcgccctcagacgagtcggatctccctttgggccgcctccccgcggtacctttaagaccaatgacttacaaggcagctgtagatcttagccactttttaaaagaaaaggggggactggaagggctaattcactcccaacgaagacaagatctgctttttgcttgtactgggtctctctggttagaccagatctgagcctgggagctctctggctaactagggaacccactgcttaagcctcaataaagcttgccttgagtgcttcaagtagtgtgtgcccgtctgttgtgtgactctggtaactagagatccctcagacccttttagtcagtgtggaaaatctctagcagtagtagttcatgtcatcttattattcagtatttataacttgcaaagaaatgaatatcagagagtgagaggaacttgtttattgcagcttataatggttacaaataaagcaatagcatcacaaatttcacaaataaagcatttttttcactgcattctagttgtggtttgtccaaactcatcaatgtatcttatcatgtctggctctagctatcccgcccctaactccgcccatcccgcccctaactccgcccagttccgcccattctccgccccatggctgactaattttttttatttatgcagaggccgaggccgcctcggcctctgagctattccagaagtagtgaggaggcttttttggaggccgctagcgtcgaccattacttattgttttagctgtcctcatgaatgtcttttcactacccatttgcttatcctgcatctctcagccttgactccactcagttctcttgcttagagataccacctttcccctgaagtgttccttccatgttttacggcgagatggtttctcctcgcctggccactcagccttagttgtctctgttgtcttatagaggtctacttgaagaaggaaaaacagggggcatggtttgactgtcctgtgagcccttcttccctgcctcccccactcacagtgacccggaatccctcgacatggcagtctagcactagtgcggccgcagatctgcttcctcgctcactgactcgctgcgctcggtcgttcggctgcggcgagcggtatcagctcactcaaaggcggtaatacggttatccacagaatcaggggataacgcaggaaagaacatgtgagcaaaaggccagcaaaaggccaggaaccgtaaaaa

SEQ ID NO: 19 - DNA, 9161 bp, synthetic construct
  misc_feature 1..9161: note = pKL-Kan-lenti-CBH-KL-BsHIV01-003
  source 1..9161: mol_type = other DNA
ggccgcgttgctggcgtttttccataggctccgcccccctgacgagcatcacaaaaatcgacgctcaagtcagaggtggcgaaacccgacaggactataaagataccaggcgtttccccctggaagctccctcgtgcgctctcctgttccgaccctgccgcttaccggatacctgtccgcctttctcccttcgggaagcgtggcgctttctcatagctcacgctgtaggtatctcagttcggtgtaggtcgttcgctccaagctgggctgtgtgcacgaaccccccgttcagcccgaccgctgcgccttatccggtaactatcgtcttgagtccaacccggtaagacacgacttatcgccactggcagcagccactggtaacaggattagcagagcgaggtatgtaggcggtgctacagagttcttgaagtggtggcctaactacggctacactagaagaacagtatttggtatctgcgctctgctgaagccagttaccttcggaaaaagagttggtagctcttgatccggcaaacaaaccaccgctggtagcggtggtttttttgtttgcaagcagcagattacgcgcagaaaaaaaggatctcaagaagatcctttgatcttttctacggggtctgacgctcagtggaacgaaaactcacgttaagggattttggtcatgaagcgcttttgaagctcggatccgaacaaacgacccaacacccgtgcgttttattctgtctttttattgccgatcccctcagaagaactcgtcaagaaggcgatagaaggcgatgcgctgcgaatcgggagcggcgataccgtaaagcacgaggaagcggtcagcccattcgccgccaagctcttcagcaatatcacgggtagccaacgctatgtcctgatagcggtccgccacacccagccggccacagtcgatgaatccagaaaagcggccattttccaccatgatattcggcaagcaggcatcgccatgggtcacgacgagatcctcgccgtcgggcatgctcgccttgagcctggcgaacagttcggctggcgcgagcccctgatgctcttcgtccagatcatcctgatcgacaagaccggcttccatccgagtacgtgctcgctcgatgcgatgtttcgcttggtggtcgaatgggcaggtagccggatcaagcgtatgcagccgccgcattgcatcagccatgatggatactttctcggcaggagcaaggtgagatgacaggagatcctgccccggcacttcgcccaatagcagccagtcccttcccgcttcagtgacaacgtcgagcacagctgcgcaaggaacgcccgtcgtggccagccacgatagccgcgctgcctcgtcttgcagttcattcagggcaccggacaggtcggtcttgacaaaaagaaccgggcgcccctgcgctgacagccggaacacggcggcatcagagcagccgattgtctgttgtgcccagtcatagccgaatagcctctccacccaagcggccggagaacctgcgtgcaatccatcttgttcaatcatgcgaaacgatcctcatcctgtctcttgatcagagcttgatcccctgcgccatcagatccttggcggcaagaaagccatccagtttactttgcagggcttcccaaccttaccagaggcctgcgccgcggccagctggctagcaattcccgggttaactctagagacattgattattgactagttattaatagtaatcaattacggggtcattagttcatagcccatatatggagttccgcgttacataacttacggtaaatggcccgcctggctgaccgcccaacgacccccgcccattgacgtcaataatgacgtatgttcccatagtaacgccaatagggactttccattgacgtcaatgggtggagtatttacggtaaactgcccacttggcagtacatcaagtgtatcatatgccaagtacgccccctattgacgtcaatgacggtaaatggcccgcctggcattatgcccagtacatgaccttatgggactttcctacttggcagtacatctacgtattagtcatcgctattaccatggtgatgcggttttggcagtacatcaatgggcgtggatagcggtttgactcacggggatttccaagtctccaccccattgacgtcaatgggagtttgttttggcaccaaaatcaacgggactttccaaaatgtcgtaacaactccgccccattgacgcaaatgggcggtaggcgtgtacggtgggaggtctatataagcagagctcgtttagtgaaccggggtctctctggttagaccagatctgagcctgggagctctctggctaactagggaacccactgcttaagcctcaataaagcttgccttgagtgcttcaagtagtgtgtgcccgtctgttgtgtgactctggtaactagagatccctcagacccttttagtcagtgtggaaaatctctagcagtggcgcccgaacagggacttgaaagcgaaagggaaaccagaggagctctctcgacgcaggactcggcttgctgaagcgcgcacggcaagaggcgaggggcggcgactggtgagtacgccaaaaattttgactagcggaggctagaaggagagagatgggtgcgagagcgtcagtattaagcgggggagaattagatcgcgatgggaaaaaattcggttaaggccagggggaaagaaaaaatataaattaaaacatatagtatgggcaagcagggagctagaacgattcgcagttaatcctggcctgttagaaacatcagaaggctgtagacaaatactgggacagctacaaccatcccttcagacaggatcagaagaacttagatcattatataatacagtagcaaccctctattgtgtgcatcaaaggatagagataaaagacaccaaggaagctttagacaagatagaggaagagcaaaacaaaagtaagaccaccgcacagcaagcggccgctgatcttcagacctggaggaggagatatgagggacaattggagaagtgaattatataaatataaagtagtaaaaattgaaccattaggagtagcacccaccaaggcaaagagaagagtggtgcagagagaaaaaagagcagtgggaataggagctttgttccttgggttcttgggagcagcaggaagcactatgggcgcagcgtcaatgacgctgacggtacaggccagacaattattgtctggtatagtgcagcagcagaacaatttgctgagggctattgaggcgcaacagcatctgttgcaactcacagtctggggcatcaagcagctccaggcaagaatcctggctgtggaaagatacctaaaggatcaacagctcctggggatttggggttgctctggaaaactcatttgcaccactgctgtgccttggaatgctagttggagtaataaatctctggaacagatttggaatcacacgacctggatggagtgggacagagaaattaacaattacacaagcttaatacactccttaattgaagaatcgcaaaaccagcaagaaaagaatgaacaagaattattggaattagataaatgggcaagtttgtggaattggtttaacataacaaattggctgtggtatataaaattattcataatgatagtaggaggcttggtaggtttaagaatagtttttgctgtactttctatagtgaatagagttaggcagggatattcaccattatcgtttcagacccacctcccaaccccgaggggacccgacaggcccgaaggaatagaagaagaaggtggagagagagacagagacagatccattcgattagtgaacggatctcgacggtatcggttaacttttaaaagaaaaggggggattggggggtacagtgcaggggaaagaatagtagacataatagcaacagacatacaaactaaagaattacaaaaacaaattacaaaaattcaaaattttatcgatcacgagactagcctcgaggcatgcctgcaggaattccgttacataacttacggtaaatggcccgcctggctgaccgcccaacgacccccgcccattgacgtcaataatgacgtatgttcccatagtaacgccaatagggactttccattgacgtcaatgggtggagtatttacggtaaactgcccacttggcagtacatcaagtgtatcatatgccaagtacgccccctattgacgtcaatgacggtaaatggcccgcctggcattatgcccagtacatgaccttatgggactttcctacttggcagtacatctacgtattagtcatcgctattaccatggtcgaggtgagccccacgttctgcttcactctccccatctcccccccctccccacccccaattttgtatttatttattttttaattattttgtgcagcgatgggggcggggggggggggggggcgcgcgccaggcggggcggggcggggcgaggggcggggcggggcgaggcggagaggtgcggcggcagccaatcagagcggcgcgctccgaaagtttccttttatggcgaggcggcggcggcggcggccctataaaaagcgaagcgcgcggcgggcgggagtcgctgcgacgctgccttcgccccgtgccccgctccgccgccgcctcgcgccgcccgccccggctctgactgaccgcgttactcccacaggtgagcgggcgggacggcccttctcctccgggctgtaattagctgagcaagaggtaagggtttaagggatggttggttggtggggtattaatgtttaattacctggagcacctgcctgaaatcactttttttcaggtaccggtcgccaccatggcgagacccctgtgcacattacttctgttgatggctaccctggcaggcgccctcgccagcgagctgacacaggaccctgccgtgtccgtggccctgaagcagaccgtgacaatcacctgcagaggcgattccctgagatcccactacgcctcctggtaccagaagaagcctggccaggcccccgtgctgctgttttacggcaagaataaccgccccagcggcatccccgatagattttccggcagcgcctccggcaacagagccagcctgacaatcaccggcgcccaggccgaggacgaggctgattactactgcagctccagagataagagcggcagcagactgtccgtgtttggcggcggcaccaagctgaccgtgctcggaggaggaggaagcggaggaggaggctcaggcggcggcggctctgaggtgaggctgagagagtccggcggcggcctggtgaagcccggaggatctctgaggctgtcctgctccgcctccggcttcgattttgacaatgcctggatgacctgggtgagacagccccctggcaagggcctggagtgggtgggaaggatcacaggccccggcgagggctggtccgtggattacgccgagtccgtgaagggcaggttcacaatctccagggataacaccaagaacaccctgtacctggagatgaacaacgtgaggacagaggataccggctactacttttgcgccagaacaggcaagtactacgacttttggttcggctacccccctggcgaggagtacttccaggattggggccagggcaccctggtcattgtgtccagcggcggcggcggcagtggcggcggcggaagcggcggcggcggctctggcggcggcggcagcggcggcggcggctccgacatcgtgatgacccagtctcctgatagcctggccgtgagcctgggcgagagagtgacaatgaactgtaagtctagccagagcctgctgtactccaccaaccagaagaattacctggcctggtatcagcagaagcctggccagtccccaaagctgctgatctattgggcatctacaagggagagcggagtgccagacagattcagcggatccggatctggaaccgacttcaccctgacaatctcctctgtgcaggccgaggacgtggccgtgtactattgccagcagtactatagctacaggacattcggcggcggcaccaagctggagatcaagcgcaccgtggccggaggaggaggatctggcggaggagggtccggcggcggcggctcccaggtgcagctgcagcagagcggaccagaggtggtgaagcctggagcctccgtgaagatgtcttgtaaggccagcggctacaccttcacatcctatgtgatccactgggtgaggcagaagccaggacagggactggactggatcggctacatcaacccttataatgatggcaccgactacgatgagaagtttaagggcaaggccaccctgacatccgataccagcacatccaccgcctatatggagctgagctccctgcggtctgaggacacagccgtgtactattgcgccagagagaaggataactacgcaaccggagcatggttcgcatattggggacagggtaccctggtcaccgtgtctagcgagcccaagagctgtgacaagacacacacctgccctccatgtccagcaccagagctgctgggagggccctccgtgttcctgtttccccctaagccaaaggatacactgatgatctccaggacaccagaggtgacctgcgtggtggtggacgtgtctcacgaggatcctgaggtgaagtttaactggtacgtggacggcgtggaggtgcacaatgccaagaccaagcctagggaggagcagtacaattctacatatcgcgtggtgagcgtgctgaccgtgctgcaccaggattggctgaacggcaaggagtataagtgcaaggtgagcaataaggccctgcctgccccaatcgagaagacaatctccaaggcaaagggacagccaagggagcctcaggtgtacaccctgccaccctctcgcgacgagctgacaaagaaccaggtgagcctgacctgtctggtgaagggcttctatcctagcgatattgccgtggagtgggagtccaatggccagccagagaacaattacaagaccacacctccagtgctggactccgatggctctttctttctgtattccaagctgacagtggacaagtctagatggcagcagggcaacgtgttttcttgtagcgtgatgcacgaggccctgcacaatcactacacccagaagtccctgtctctgagccccggcaagggcggaggaggaagcggaggaggcggctctggcggaggaggttccggaggaggcggaagcggcggaggaggctcttgggagcagaagatcgaggagctgctgaagaaggccgaggagcagcagaagaagaatgaggaggagctgaagaagctggagaagtaggtcgacaatcaacctctggattacaaaatttgtgaaagattgactggtattcttaactatgttgctccttttacgctatgtggatacgctgctttaatgcctttgtatcatgctattgcttcccgtatggctttcattttctcctccttgtataaatcctggttgctgtctctttatgaggagttgtggcccgttgtcaggcaacgtggcgtggtgtgcactgtgtttgctgacgcaacccccactggttggggcattgccaccacctgtcagctcctttccgggactttcgctttccccctccctattgccacggcggaactcatcgccgcctgccttgcccgctgctggacaggggctcggctgttgggcactgacaattccgtggtgttgtcggggaagctgacgtcctttccatggctgctcgcctgtgttgccacctggattctgcgcgggacgtccttctgctacgtcccttcggccctcaatccagcggaccttccttcccgcggcctgctgccggctctgcggcctcttccgcgtcttcgccttcgccctcagacgagtcggatctccctttgggccgcctccccgcggtacctttaagaccaatgacttacaaggcagctgtagatcttagccactttttaaaagaaaaggggggactggaagggctaattcactcccaacgaagacaagatctgctttttgcttgtactgggtctctctggttagaccagatctgagcctgggagctctctggctaactagggaacccactgcttaagcctcaataaagcttgccttgagtgcttcaagtagtgtgtgcccgtctgttgtgtgactctggtaactagagatccctcagacccttttagtcagtgtggaaaatctctagcagtagtagttcatgtcatcttattattcagtatttataacttgcaaagaaatgaatatcagagagtgagaggaacttgtttattgcagcttataatggttacaaataaagcaatagcatcacaaatttcacaaataaagcatttttttcactgcattctagttgtggtttgtccaaactcatcaatgtatcttatcatgtctggctctagctatcccgcccctaactccgcccatcccgcccctaactccgcccagttccgcccattctccgccccatggctgactaattttttttatttatgcagaggccgaggccgcctcggcctctgagctattccagaagtagtgaggaggcttttttggaggccgctagcgtcgaccattacttattgttttagctgtcctcatgaatgtcttttcactacccatttgcttatcctgcatctctcagccttgactccactcagttctcttgcttagagataccacctttcccctgaagtgttccttccatgttttacggcgagatggtttctcctcgcctggccactcagccttagttgtctctgttgtcttatagaggtctacttgaagaaggaaaaacagggggcatggtttgactgtcctgtgagcccttcttccctgcctcccccactcacagtgacccggaatccctcgacatggcagtctagcactagtgcggccgcagatctgcttcctcgctcactgactcgctgcgctcggtcgttcggctgcggcgagcggtatcagctcactcaaaggcggtaatacggttatccacagaatcaggggataacgcaggaaagaacatgtgagcaaaaggccagcaaaaggccaggaaccgtaaaaa

SEQ ID NO: 20 - DNA, 7022 bp, synthetic construct
  misc_feature 1..7022: note = pAAV-MCS-CMV-EGFP(reverse)
  source 1..7022: mol_type = other DNA
acatgtgagcaaaaggccagcaaaaggccaggaaccgtaaaaaggccgcgttgctggcgtttttccataggctccgcccccctgacgagcatcacaaaaatcgacgctcaagtcagaggtggcgaaacccgacaggactataaagataccaggcgtttccccctggaagctccctcgtgcgctctcctgttccgaccctgccgcttaccggatacctgtccgcctttctcccttcgggaagcgtggcgctttctcatagctcacgctgtaggtatctcagttcggtgtaggtcgttcgctccaagctgggctgtgtgcacgaaccccccgttcagcccgaccgctgcgccttatccggtaactatcgtcttgagtccaacccggtaagacacgacttatcgccactggcagcagccactggtaacaggattagcagagcgaggtatgtaggcggtgctacagagttcttgaagtggtggcctaactacggctacactagaaggacagtatttggtatctgcgctctgctgaagccagttaccttcggaaaaagagttggtagctcttgatccggcaaacaaaccaccgctggtagcggtggtttttttgtttgcaagcagcagattacgcgcagaaaaaaaggatctcaagaagatcctttgatcttttctacggggtctgacgctcagtggaacgaaaactcacgttaagggattttggtcatgagattatcaaaaaggatcttcacctagatccttttaaattaaaaatgaagttttaaatcaatctaaagtatatatgagtaaacttggtctgacagttaccaatgcttaatcagtgaggcacctatctcagcgatctgtctatttcgttcatccatagttgcctgactccccgtcgtgtagataactacgatacgggagggcttaccatctggccccagtgctgcaatgataccgcgagacccacgctcaccggctccagatttatcagcaataaaccagccagccggaagggccgagcgcagaagtggtcctgcaactttatccgcctccatccagtctattaattgttgccgggaagctagagtaagtagttcgccagttaatagtttgcgcaacgttgttgccattgctacaggcatcgtggtgtcacgctcgtcgtttggtatggcttcattcagctccggttcccaacgatcaaggcgagttacatgatcccccatgttgtgcaaaaaagcggttagctccttcggtcctccgatcgttgtcagaagtaagttggccgcagtgttatcactcatggttatggcagcactgcataattctcttactgtcatgccatccgtaagatgcttttctgtgactggtgagtactcaaccaagtcattctgagaatagtgtatgcggcgaccgagttgctcttgcccggcgtcaatacgggataataccgcgccacatagcagaactttaaaagtgctcatcattggaaaacgttcttcggggcgaaaactctcaaggatcttaccgctgttgagatccagttcgatgtaacccactcgtgcacccaactgatcttcagcatcttttactttcaccagcgtttctgggtgagcaaaaacaggaaggcaaaatgccgcaaaaaagggaataagggcgacacggaaatgttgaatactcatactcttcctttttcaatattattgaagcatttatcagggttattgtctcatgagcggatacatatttgaatgtatttagaaaaataaacaaataggggttccgcgcacatttccccgaaaagtgccacctgacgtctaagaaaccattattatcatgacattaacctataaaaataggcgtatcacgaggccctttcgtctcgcgcgtttcggtgatgacggtgaaaacctctgacacatgcagctcccggagacggtcacagcttgtctgtaagcggatgccgggagcagacaagcccgtcagggcgcgtcagcgggtgttggcgggtgtcggggctggcttaactatgcggcatcagagcagattgtactgagagtgcaccataaaattgtaaacgttaatattttgttaaaattcgcgttaaatttttgttaaatcagctcattttttaaccaataggccgaaatcggcaaaatcccttataaatcaaaagaatagcccgagatagggttgagtgttgttccagtttggaacaagagtccactattaaagaacgtggactccaacgtcaaagggcgaaaaaccgtctatcagggcgatggcccactacgtgaaccatcacccaaatcaagttttttggggtcgaggtgccgtaaagcactaaatcggaaccctaaagggagcccccgatttagagcttgacggggaaagccggcgaacgtggcgagaaaggaagggaagaaagcgaaaggagcgggcgctagggcgctggcaagtgtagcggtcacgctgcgcgtaaccaccacacccgccgcgcttaatgcgccgctacagggcgcgtactatggttgctttgacgtatgcggtgtgaaataccgcacagatgcgtaaggagaaaataccgcatcaggcgcccctgcaggcagctgcgcgctcgctcgctcactgaggccgcccgggcaaagcccgggcgtcgggcgacctttggtcgcccggcctcagtgagcgagcgagcgcgcagagagggagtggccaactccatcactaggggttcctacgcgtcgttacataacttacggtaaatggcccgcctggctgaccgcccaacgacccccgcccattgacgtcaataatgacgtatgttcccatagtaacgccaatagggactttccattgacgtcaatgggtggagtatttacggtaaactgcccacttggcagtacatcaagtgtatcatatgccaagtacgccccctattgacgtcaatgacggtaaatggcccgcctggcattatgcccagtacatgaccttatgggactttcctacttggcagtacatctacgtattagtcatcgctattaccatggtcgaggtgagccccacgttctgcttcactctccccatctcccccccctccccacccccaattttgtatttatttattttttaattattttgtgcagcgatgggggcggggggggggggggggcgcgcgccaggcggggcggggcggggcgaggggcggggcggggcgaggcggagaggtgcggcggcagccaatcagagcggcgcgctccgaaagtttccttttatggcgaggcggcggcggcggcggccctataaaaagcgaagcgcgcggcgggcgggagtcgctgcgacgctgccttcgccccgtgccccgctccgccgccgcctcgcgccgcccgccccggctctgactgaccgcgttactcccacaggtgagcgggcgggacggcccttctcctccgggctgtaattagctgagcaagaggtaagggtttaagggatggttggttggtggggtattaatgtttaattacctggagcacctgcctgaaatcactttttttcaggtaccggtcgccaccatggcgagacccctgtgcacattacttctgttgatggctaccctggcaggcgccctcgccagcgagctgacacaggaccctgccgtgtccgtggccctgaagcagaccgtgacaatcacctgcagaggcgattccctgagatcccactacgcctcctggtaccagaagaagcctggccaggcccccgtgctgctgttttacggcaagaataaccgccccagcggcatccccgatagattttccggcagcgcctccggcaacagagccagcctgacaatcaccggcgcccaggccgaggacgaggctgattactactgcagctccagagataagagcggcagcagactgtccgtgtttggcggcggcaccaagctgaccgtgctcggaggaggaggaagcggaggaggaggctcaggcggcggcggctctgaggtgaggctgagagagtccggcggcggcctggtgaagcccggaggatctctgaggctgtcctgctccgcctccggcttcgattttgacaatgcctggatgacctgggtgagacagccccctggcaagggcctggagtgggtgggaaggatcacaggccccggcgagggctggtccgtggattacgccgagtccgtgaagggcaggttcacaatctccagggataacaccaagaacaccctgtacctggagatgaacaacgtgaggacagaggataccggctactacttttgcgccagaacaggcaagtactacgacttttggttcggctacccccctggcgaggagtacttccaggattggggccagggcaccctggtcattgtgtccagcggcggcggcggcagtggcggcggcggaagcggcggcggcggctctggcggcggcggcagcggcggcggcggctccgacatcgtgatgacccagtctcctgatagcctggccgtgagcctgggcgagagagtgacaatgaactgtaagtctagccagagcctgctgtactccaccaaccagaagaattacctggcctggtatcagcagaagcctggccagtccccaaagctgctgatctattgggcatctacaagggagagcggagtgccagacagattcagcggatccggatctggaaccgacttcaccctgacaatctcctctgtgcaggccgaggacgtggccgtgtactattgccagcagtactatagctacaggacattcggcggcggcaccaagctggagatcaagcgcaccgtggccggaggaggaggatctggcggaggagggtccggcggcggcggctcccaggtgcagctgcagcagagcggaccagaggtggtgaagcctggagcctccgtgaagatgtcttgtaaggccagcggctacaccttcacatcctatgtgatccactgggtgaggcagaagccaggacagggactggactggatcggctacatcaacccttataatgatggcaccgactacgatgagaagtttaagggcaaggccaccctgacatccgataccagcacatccaccgcctatatggagctgagctccctgcggtctgaggacacagccgtgtactattgcgccagagagaaggataactacgcaaccggagcatggttcgcatattggggacagggtaccctggtcaccgtgtctagcgagcccaagagctgtgacaagacacacacctgccctccatgtccagcaccagagctgctgggagggccctccgtgttcctgtttccccctaagccaaaggatacactgatgatctccaggacaccagaggtgacctgcgtggtggtggacgtgtctcacgaggatcctgaggtgaagtttaactggtacgtggacggcgtggaggtgcacaatgccaagaccaagcctagggaggagcagtacaattctacatatcgcgtggtgagcgtgctgaccgtgctgcaccaggattggctgaacggcaaggagtataagtgcaaggtgagcaataaggccctgcctgccccaatcgagaagacaatctccaaggcaaagggacagccaagggagcctcaggtgtacaccctgccaccctctcgcgacgagctgacaaagaaccaggtgagcctgacctgtctggtgaagggcttctatcctagcgatattgccgtggagtgggagtccaatggccagccagagaacaattacaagaccacacctccagtgctggactccgatggctctttctttctgtattccaagctgacagtggacaagtctagatggcagcagggcaacgtgttttcttgtagcgtgatgcacgaggccctgcacaatcactacacccagaagtccctgtctctgagccccggcaagggcggaggaggaagcggaggaggcggctctggcggaggaggttccggaggaggcggaagcggcggaggaggctctctgctggagcaggagaacaaggagcagcagaatcagagcgaggagatcctgtcccacatcctgtccacatacaacaatatcgagagagattgggagatgtggtaggtcgacaatcaacctctggattacaaaatttgtgaaagattgactggtattcttaactatgttgctccttttacgctatgtggatacgctgctttaatgcctttgtatcatgctattgcttcccgtatggctttcattttctcctccttgtataaatcctggttgctgtctctttatgaggagttgtggcccgttgtcaggcaacgtggcgtggtgtgcactgtgtttgctgacgcaacccccactggttggggcattgccaccacctgtcagctcctttccgggactttcgctttccccctccctattgccacggcggaactcatcgccgcctgccttgcccgctgctggacaggggctcggctgttgggcactgacaattccgtggtgttgtcggggaagctgacgtcctttccatggctgctcgcctgtgttgccacctggattctgcgcgggacgtccttctgctacgtcccttcggccctcaatccagcggaccttccttcccgcggcctgctgccggctctgcggcctcttccgcgtcttcgccttcgccctcagacgagtcggatctccctttgggccgcctccccgcgaattcgtttatttgtgaaatttgtgatgctattgctttatttgtaaccatctagctttatttgtgaaatttgtgatgctattgctttatttgtaaccattataagctgcaataaacaagttaacaacaacaattgcattcattttatgtttcaggttcagggggagatgtgggaggttttttaaagtttaaacaggaacccctagtgatggagttggccactccctctctgcgcgctcgctcgctcactgaggccgggcgaccaaaggtcgcccgacgcccgggcggcctcagtgagcgagcgagcgcgcagctgcctgcagg

SEQ ID NO: 21 - DNA, 6845 bp, synthetic construct
  misc_feature 1..6845: note = pAAV-CBH-KL-BsHIV01-WPRE
  source 1..6845: mol_type = other DNA
acatgtgagcaaaaggccagcaaaaggccaggaaccgtaaaaaggccgcgttgctggcgtttttccataggctccgcccccctgacgagcatcacaaaaatcgacgctcaagtcagaggtggcgaaacccgacaggactataaagataccaggcgtttccccctggaagctccctcgtgcgctctcctgttccgaccctgccgcttaccggatacctgtccgcctttctcccttcgggaagcgtggcgctttctcatagctcacgctgtaggtatctcagttcggtgtaggtcgttcgctccaagctgggctgtgtgcacgaaccccccgttcagcccgaccgctgcgccttatccggtaactatcgtcttgagtccaacccggtaagacacgacttatcgccactggcagcagccactggtaacaggattagcagagcgaggtatgtaggcggtgctacagagttcttgaagtggtggcctaactacggctacactagaaggacagtatttggtatctgcgctctgctgaagccagttaccttcggaaaaagagttggtagctcttgatccggcaaacaaaccaccgctggtagcggtggtttttttgtttgcaagcagcagattacgcgcagaaaaaaaggatctcaagaagatcctttgatcttttctacggggtctgacgctcagtggaacgaaaactcacgttaagggattttggtcatgagattatcaaaaaggatcttcacctagatccttttaaattaaaaatgaagttttaaatcaatctaaagtatatatgagtaaacttggtctgacagttaccaatgcttaatcagtgaggcacctatctcagcgatctgtctatttcgttcatccatagttgcctgactccccgtcgtgtagataactacgatacgggagggcttaccatctggccccagtgctgcaatgataccgcgagacccacgctcaccggctccagatttatcagcaataaaccagccagccggaagggccgagcgcagaagtggtcctgcaactttatccgcctccatccagtctattaattgttgccgggaagctagagtaagtagttcgccagttaatagtttgcgcaacgttgttgccattgctacaggcatcgtggtgtcacgctcgtcgtttggtatggcttcattcagctccggttcccaacgatcaaggcgagttacatgatcccccatgttgtgcaaaaaagcggttagctccttcggtcctccgatcgttgtcagaagtaagttggccgcagtgttatcactcatggttatggcagcactgcataattctcttactgtcatgccatccgtaagatgcttttctgtgactggtgagtactcaaccaagtcattctgagaatagtgtatgcggcgaccgagttgctcttgcccggcgtcaatacgggataataccgcgccacatagcagaactttaaaagtgctcatcattggaaaacgttcttcggggcgaaaactctcaaggatcttaccgctgttgagatccagttcgatgtaacccactcgtgcacccaactgatcttcagcatcttttactttcaccagcgtttctgggtgagcaaaaacaggaaggcaaaatgccgcaaaaaagggaataagggcgacacggaaatgttgaatactcatactcttcctttttcaatattattgaagcatttatcagggttattgtctcatgagcggatacatatttgaatgtatttagaaaaataaacaaataggggttccgcgcacatttccccgaaaagtgccacctgacgtctaagaaaccattattatcatgacattaacctataaaaataggcgtatcacgaggccctttcgtctcgcgcgtttcggtgatgacggtgaaaacctctgacacatgcagctcccggagacggtcacagcttgtctgtaagcggatgccgggagcagacaagcccgtcagggcgcgtcagcgggtgttggcgggtgtcggggctggcttaactatgcggcatcagagcagattgtactgagagtgcaccataaaattgtaaacgttaatattttgttaaaattcgcgttaaatttttgttaaatcagctcattttttaaccaataggccgaaatcggcaaaatcccttataaatcaaaagaatagcccgagatagggttgagtgttgttccagtttggaacaagagtccactattaaagaacgtggactccaacgtcaaagggcgaaaaaccgtctatcagggcgatggcccactacgtgaaccatcacccaaatcaagttttttggggtcgaggtgccgtaaagcactaaatcggaaccctaaagggagcccccgatttagagcttgacggggaaagccggcgaacgtggcgagaaaggaagggaagaaagcgaaaggagcgggcgctagggcgctggcaagtgtagcggtcacgctgcgcgtaaccaccacacccgccgcgcttaatgcgccgctacagggcgcgtactatggttgctttgacgtatgcggtgtgaaataccgcacagatgcgtaaggagaaaataccgcatcaggcgcccctgcaggcagctgcgcgctcgctcgctcactgaggccgcccgggcaaagcccgggcgtcgggcgacctttggtcgcccggcctcagtgagcgagcgagcgcgcagagagggagtggccaactccatcactaggggttcctacgcgtcgttacataacttacggtaaatggcccgcctggctgaccgcccaacgacccccgcccattgacgtcaataatgacgtatgttcccatagtaacgccaatagggactttccattgacgtcaatgggtggagtatttacggtaaactgcccacttggcagtacatcaagtgtatcatatgccaagtacgccccctattgacgtcaatgacggtaaatggcccgcctggcattatgcccagtacatgaccttatgggactttcctacttggcagtacatctacgtattagtcatcgctattaccatggtcgaggtgagccccacgttctgcttcactctccccatctcccccccctccccacccccaattttgtatttatttattttttaattattttgtgcagcgatgggggcggggggggggggggggcgcgcgccaggcggggcggggcggggcgaggggcggggcggggcgaggcggagaggtgcggcggcagccaatcagagcggcgcgctccgaaagtttccttttatggcgaggcggcggcggcggcggccctataaaaagcgaagcgcgcggcgggcgggagtcgctgcgacgctgccttcgccccgtgccccgctccgccgccgcctcgcgccgcccgccccggctctgactgaccgcgttactcccacaggtgagcgggcgggacggcccttctcctccgggctgtaattagctgagcaagaggtaagggtttaagggatggttggttggtggggtattaatgtttaattacctggagcacctgcctgaaatcactttttttcaggtaccggtcgccaccatggcgagacccctgtgcacattacttctgttgatggctaccctggcaggcgccctcgccagcgagctgacacaggaccctgccgtgtccgtggccctgaagcagaccgtgacaatcacctgcagaggcgattccctgagatcccactacgcctcctggtaccagaagaagcctggccaggcccccgtgctgctgttttacggcaagaataaccgccccagcggcatccccgatagattttccggcagcgcctccggcaacagagccagcctgacaatcaccggcgcccaggccgaggacgaggctgattactactgcagctccagagataagagcggcagcagactgtccgtgtttggcggcggcaccaagctgaccgtgctcggaggaggaggaagcggaggaggaggctcaggcggcggcggctctgaggtgaggctgagagagtccggcggcggcctggtgaagcccggaggatctctgaggctgtcctgctccgcctccggcttcgattttgacaatgcctggatgacctgggtgagacagccccctggcaagggcctggagtgggtgggaaggatcacaggccccggcgagggctggtccgtggattacgccgagtccgtgaagggcaggttcacaatctccagggataacaccaagaacaccctgtacctggagatgaacaacgtgaggacagaggataccggctactacttttgcgccagaacaggcaagtactacgacttttggttcggctacccccctggcgaggagtacttccaggattggggccagggcaccctggtcattgtgtccagcggcggcggcggcagtggcggcggcggaagcggcggcggcggctctggcggcggcggcagcggcggcggcggctccgacatcgtgatgacccagtctcctgatagcctggccgtgagcctgggcgagagagtgacaatgaactgtaagtctagccagagcctgctgtactccaccaaccagaagaattacctggcctggtatcagcagaagcctggccagtccccaaagctgctgatctattgggcatctacaagggagagcggagtgccagacagattcagcggatccggatctggaaccgacttcaccctgacaatctcctctgtgcaggccgaggacgtggccgtgtactattgccagcagtactatagctacaggacattcggcggcggcaccaagctggagatcaagcgcaccgtggccggaggaggaggatctggcggaggagggtccggcggcggcggctcccaggtgcagctgcagcagagcggaccagaggtggtgaagcctggagcctccgtgaagatgtcttgtaaggccagcggctacaccttcacatcctatgtgatccactgggtgaggcagaagccaggacagggactggactggatcggctacatcaacccttataatgatggcaccgactacgatgagaagtttaagggcaaggccaccctgacatccgataccagcacatccaccgcctatatggagctgagctccctgcggtctgaggacacagccgtgtactattgcgccagagagaaggataactacgcaaccggagcatggttcgcatattggggacagggtaccctggtcaccgtgtctagcgagcccaagagctgtgacaagacacacacctgccctccatgtccagcaccagagctgctgggagggccctccgtgttcctgtttccccctaagccaaaggatacactgatgatctccaggacaccagaggtgacctgcgtggtggtggacgtgtctcacgaggatcctgaggtgaagtttaactggtacgtggacggcgtggaggtgcacaatgccaagaccaagcctagggaggagcagtacaattctacatatcgcgtggtgagcgtgctgaccgtgctgcaccaggattggctgaacggcaaggagtataagtgcaaggtgagcaataaggccctgcctgccccaatcgagaagacaatctccaaggcaaagggacagccaagggagcctcaggtgtacaccctgccaccctctcgcgacgagctgacaaagaaccaggtgagcctgacctgtctggtgaagggcttctatcctagcgatattgccgtggagtgggagtccaatggccagccagagaacaattacaagaccacacctccagtgctggactccgatggctctttctttctgtattccaagctgacagtggacaagtctagatggcagcagggcaacgtgttttcttgtagcgtgatgcacgaggccctgcacaatcactacacccagaagtccctgtctctgagccccggcaagtaggtcgacaatcaacctctggattacaaaatttgtgaaagattgactggtattcttaactatgttgctccttttacgctatgtggatacgctgctttaatgcctttgtatcatgctattgcttcccgtatggctttcattttctcctccttgtataaatcctggttgctgtctctttatgaggagttgtggcccgttgtcaggcaacgtggcgtggtgtgcactgtgtttgctgacgcaacccccactggttggggcattgccaccacctgtcagctcctttccgggactttcgctttccccctccctattgccacggcggaactcatcgccgcctgccttgcccgctgctggacaggggctcggctgttgggcactgacaattccgtggtgttgtcggggaagctgacgtcctttccatggctgctcgcctgtgttgccacctggattctgcgcgggacgtccttctgctacgtcccttcggccctcaatccagcggaccttccttcccgcggcctgctgccggctctgcggcctcttccgcgtcttcgccttcgccctcagacgagtcggatctccctttgggccgcctccccgcgaattcgtttatttgtgaaatttgtgatgctattgctttatttgtaaccatctagctttatttgtgaaatttgtgatgctattgctttatttgtaaccattataagctgcaataaacaagttaacaacaacaattgcattcattttatgtttcaggttcagggggagatgtgggaggttttttaaagtttaaacaggaacccctagtgatggagttggccactccctctctgcgcgctcgctcgctcactgaggccgggcgaccaaaggtcgcccgacgcccgggcggcctcagtgagcgagcgagcgcgcagctgcctgcagg

SEQ ID NO: 22 - DNA, 6955 bp, synthetic construct
  misc_feature 1..6955: note = pAAV-CBH-KL-BsHIV01-003-WPRE
  source 1..6955: mol_type = other DNA
acatgtgagcaaaaggccagcaaaaggccaggaaccgtaaaaaggccgcgttgctggcgtttttccataggctccgcccccctgacgagcatcacaaaaatcgacgctcaagtcagaggtggcgaaacccgacaggactataaagataccaggcgtttccccctggaagctccctcgtgcgctctcctgttccgaccctgccgcttaccggatacctgtccgcctttctcccttcgggaagcgtggcgctttctcatagctcacgctgtaggtatctcagttcggtgtaggtcgttcgctccaagctgggctgtgtgcacgaaccccccgttcagcccgaccgctgcgccttatccggtaactatcgtcttgagtccaacccggtaagacacgacttatcgccactggcagcagccactggtaacaggattagcagagcgaggtatgtaggcggtgctacagagttcttgaagtggtggcctaactacggctacactagaaggacagtatttggtatctgcgctctgctgaagccagttaccttcggaaaaagagttggtagctcttgatccggcaaacaaaccaccgctggtagcggtggtttttttgtttgcaagcagcagattacgcgcagaaaaaaaggatctcaagaagatcctttgatcttttctacggggtctgacgctcagtggaacgaaaactcacgttaagggattttggtcatgagattatcaaaaaggatcttcacctagatccttttaaattaaaaatgaagttttaaatcaatctaaagtatatatgagtaaacttggtctgacagttaccaatgcttaatcagtgaggcacctatctcagcgatctgtctatttcgttcatccatagttgcctgactccccgtcgtgtagataactacgatacgggagggcttaccatctggccccagtgctgcaatgataccgcgagacccacgctcaccggctccagatttatcagcaataaaccagccagccggaagggccgagcgcagaagtggtcctgcaactttatccgcctccatccagtctattaattgttgccgggaagctagagtaagtagttcgccagttaatagtttgcgcaacgttgttgccattgctacaggcatcgtggtgtcacgctcgtcgtttggtatggcttcattcagctccggttcccaacgatcaaggcgagttacatgatcccccatgttgtgcaaaaaagcggttagctccttcggtcctccgatcgttgtcagaagtaagttggccgcagtgttatcactcatggttatggcagcactgcataattctcttactgtcatgccatccgtaagatgcttttctgtgactggtgagtactcaaccaagtcattctgagaatagtgtatgcggcgaccgagttgctcttgcccggcgtcaatacgggataataccgcgccacatagcagaactttaaaagtgctcatcattggaaaacgttcttcggggcgaaaactctcaaggatcttaccgctgttgagatccagttcgatgtaacccactcgtgcacccaactgatcttcagcatcttttactttcaccagcgtttctgggtgagcaaaaacaggaaggcaaaatgccgcaaaaaagggaataagggcgacacggaaatgttgaatactcatactcttcctttttcaatattattgaagcatttatcagggttattgtctcatgagcggatacatatttgaatgtatttagaaaaataaacaaataggggttccgcgcacatttccccgaaaagtgccacctgacgtctaagaaaccattattatcatgacattaacctataaaaataggcgtatcacgaggccctttcgtctcgcgcgtttcggtgatgacggtgaaaacctctgacacatgcagctcccggagacggtcacagcttgtctgtaagcggatgccgggagcagacaagcccgtcagggcgcgtcagcgggtgttggcgggtgtcggggctggcttaactatgcggcatcagagcagattgtactgagagtgcaccataaaattgtaaacgttaatattttgttaaaattcgcgttaaatttttgttaaatcagctcattttttaaccaataggccgaaatcggcaaaatcccttataaatcaaaagaatagcccgagatagggttgagtgttgttccagtttggaacaagagtccactattaaagaacgtggactccaacgtcaaagggcgaaaaaccgtctatcagggcgatggcccactacgtgaaccatcacccaaatcaagttttttggggtcgaggtgccgtaaagcactaaatcggaaccctaaagggagcccccgatttagagcttgacggggaaagccggcgaacgtggcgagaaaggaagggaagaaagcgaaaggagcgggcgctagggcgctggcaagtgtagcggtcacgctgcgcgtaaccaccacacccgccgcgcttaatgcgccgctacagggcgcgtactatggttgctttgacgtatgcggtgtgaaataccgcacagatgcgtaaggagaaaataccgcatcaggcgcccctgcaggcagctgcgcgctcgctcgctcactgaggccgcccgggcaaagcccgggcgtcgggcgacctttggtcgcccggcctcagtgagcgagcgagcgcgcagagagggagtggccaactccatcactaggggttcctacgcgtcgttacataacttacggtaaatggcccgcctggctgaccgcccaacgacccccgcccattgacgtcaataatgacgtatgttcccatagtaacgccaatagggactttccattgacgtcaatgggtggagtatttacggtaaactgcccacttggcagtacatcaagtgtatcatatgccaagtacgccccctattgacgtcaatgacggtaaatggcccgcctggcattatgcccagtacatgaccttatgggactttcctacttggcagtacatctacgtattagtcatcgctattaccatggtcgaggtgagccccacgttctgcttcactctccccatctcccccccctccccacccccaattttgtatttatttattttttaattattttgtgcagcgatgggggcggggggggggggggggcgcgcgccaggcggggcggggcggggcgaggggcggggcggggcgaggcggagaggtgcggcggcagccaatcagagcggcgcgctccgaaagtttccttttatggcgaggcggcggcggcggcggccctataaaaagcgaagcgcgcggcgggcgggagtcgctgcgacgctgccttcgccccgtgccccgctccgccgccgcctcgcgccgcccgccccggctctgactgaccgcgttactcccacaggtgagcgggcgggacggcccttctcctccgggctgtaattagctgagcaagaggtaagggtttaagggatggttggttggtggggtattaatgtttaattacctggagcacctgcctgaaatcactttttttcaggtaccggtcgccaccatggcgagacccctgtgcacattacttctgttgatggctaccctggcaggcgccctcgccagcgagctgacacaggaccctgccgtgtccgtggccctgaagcagaccgtgacaatcacctgcagaggcgattccctgagatcccactacgcctcctggtaccagaagaagcctggccaggcccccgtgctgctgttttacggcaagaataaccgccccagcggcatccccgatagattttccggcagcgcctccggcaacagagccagcctgacaatcaccggcgcccaggccgaggacgaggctgattactactgcagctccagagataagagcggcagcagactgtccgtgtttggcggcggcaccaagctgaccgtgctcggaggaggaggaagcggaggaggaggctcaggcggcggcggctctgaggtgaggctgagagagtccggcggcggcctggtgaagcccggaggatctctgaggctgtcctgctccgcctccggcttcgattttgacaatgcctggatgacctgggtgagacagccccctggcaagggcctggagtgggtgggaaggatcacaggccccggcgagggctggtccgtggattacgccgagtccgtgaagggcaggttcacaatctccagggataacaccaagaacaccctgtacctggagatgaacaacgtgaggacagaggataccggctactacttttgcgccagaacaggcaagtactacgacttttggttcggctacccccctggcgaggagtacttccaggattggggccagggcaccctggtcattgtgtccagcggcggcggcggcagtggcggcggcggaagcggcggcggcggctctggcggcggcggcagcggcggcggcggctccgacatcgtgatgacccagtctcctgatagcctggccgtgagcctgggcgagagagtgacaatgaactgtaagtctagccagagcctgctgtactccaccaaccagaagaattacctggcctggtatcagcagaagcctggccagtccccaaagctgctgatctattgggcatctacaagggagagcggagtgccagacagattcagcggatccggatctggaaccgacttcaccctgacaatctcctctgtgcaggccgaggacgtggccgtgtactattgccagcagtactatagctacaggacattcggcggcggcaccaagctggagatcaagcgcaccgtggccggaggaggaggatctggcggaggagggtccggcggcggcggctcccaggtgcagctgcagcagagcggaccagaggtggtgaagcctggagcctccgtgaagatgtcttgtaaggccagcggctacaccttcacatcctatgtgatccactgggtgaggcagaagccaggacagggactggactggatcggctacatcaacccttataatgatggcaccgactacgatgagaagtttaagggcaaggccaccctgacatccgataccagcacatccaccgcctatatggagctgagctccctgcggtctgaggacacagccgtgtactattgcgccagagagaaggataactacgcaaccggagcatggttcgcatattggggacagggtaccctggtcaccgtgtctagcgagcccaagagctgtgacaagacacacacctgccctccatgtccagcaccagagctgctgggagggccctccgtgttcctgtttccccctaagccaaaggatacactgatgatctccaggacaccagaggtgacctgcgtggtggtggacgtgtctcacgaggatcctgaggtgaagtttaactggtacgtggacggcgtggaggtgcacaatgccaagaccaagcctagggaggagcagtacaattctacatatcgcgtggtgagcgtgctgaccgtgctgcaccaggattggctgaacggcaaggagtataagtgcaaggtgagcaataaggccctgcctgccccaatcgagaagacaatctccaaggcaaagggacagccaagggagcctcaggtgtacaccctgccaccctctcgcgacgagctgacaaagaaccaggtgagcctgacctgtctggtgaagggcttctatcctagcgatattgccgtggagtgggagtccaatggccagccagagaacaattacaagaccacacctccagtgctggactccgatggctctttctttctgtattccaagctgacagtggacaagtctagatggcagcagggcaacgtgttttcttgtagcgtgatgcacgaggccctgcacaatcactacacccagaagtccctgtctctgagccccggcaagggcggaggaggaagcggaggaggcggctctggcggaggaggttccggaggaggcggaagcggcggaggaggctcttgggagcagaagatcgaggagctgctgaagaaggccgaggagcagcagaagaagaatgaggaggagctgaagaagctggagaagtaggtcgacaatcaacctctggattacaaaatttgtgaaagattgactggtattcttaactatgttgctccttttacgctatgtggatacgctgctttaatgcctttgtatcatgctattgcttcccgtatggctttcattttctcctccttgtataaatcctggttgctgtctctttatgaggagttgtggcccgttgtcaggcaacgtggcgtggtgtgcactgtgtttgctgacgcaacccccactggttggggcattgccaccacctgtcagctcctttccgggactttcgctttccccctccctattgccacggcggaactcatcgccgcctgccttgcccgctgctggacaggggctcggctgttgggcactgacaattccgtggtgttgtcggggaagctgacgtcctttccatggctgctcgcctgtgttgccacctggattctgcgcgggacgtccttctgctacgtcccttcggccctcaatccagcggaccttccttcccgcggcctgctgccggctctgcggcctcttccgcgtcttcgccttcgccctcagacgagtcggatctccctttgggccgcctccccgcgaattcgtttatttgtgaaatttgtgatgctattgctttatttgtaaccattataagctgcaataaacaagttaacaacaacaattgcattcattttatgtttcaggttcagggggagatgtgggaggttttttaaagtttaaacaggaacccctagtgatggagttggccactccctctctgcgcgctcgctcgctcactgaggccgggcgaccaaaggtcgcccgacgcccgggcggcctcagtgagcgagcgagcgcgcagctgcctgcagg

SEQ ID NO: 23 - DNA, 7022 bp, synthetic construct; identical to SEQ ID NO: 20
  misc_feature 1..7022: note = pAAV-CBH-KL-BsHIV01-C34-WPRE
  source 1..7022: mol_type = other DNA

SEQ ID NO: 24 - DNA, 7028 bp, synthetic construct
  misc_feature 1..7028: note = pAAV-CBH-KL-BsHIV01-T20-WPRE
  source 1..7028: mol_type = other DNA
acatgtgagcaaaaggccagcaaaaggccaggaaccgtaaaaaggccgcgttgctggcgtttttccataggctccgcccccctgacgagcatcacaaaaatcgacgctcaagtcagaggtggcgaaacccgacaggactataaagataccaggcgtttccccctggaagctccctcgtgcgctctcctgttccgaccctgccgcttaccggatacctgtccgcctttctcccttcgggaagcgtggcgctttctcatagctcacgctgtaggtatctcagttcggtgtaggtcgttcgctccaagctgggctgtgtgcacgaaccccccgttcagcccgaccgctgcgccttatccggtaactatcgtcttgagtccaacccggtaagacacgacttatcgccactggcagcagccactggtaacaggattagcagagcgaggtatgtaggcggtgctacagagttcttgaagtggtggcctaactacggctacactagaaggacagtatttggtatctgcgctctgctgaagccagttaccttcggaaaaagagttggtagctcttgatccggcaaacaaaccaccgctggtagcggtggtttttttgtttgcaagcagcagattacgcgcagaaaaaaaggatctcaagaagatcctttgatcttttctacggggtctgacgctcagtggaacgaaaactcacgttaagggattttggtcatgagattatcaaaaaggatcttcacctagatccttttaaattaaaaatgaagttttaaatcaatctaaagtatatatgagtaaacttggtctgacagttaccaatgcttaatcagtgaggcacctatctcagcgatctgtctatttcgttcatccatagttgcctgactccccgtcgtgtagataactacgatacgggagggcttaccatctggccccagtgctgcaatgataccgcgagacccacgctcaccggctccagatttatcagcaataaaccagccagccggaagggccgagcgcagaagtggtcctgcaactttatccgcctccatccagtctattaattgttgccgggaagctagagtaagtagttcgccagttaatagtttgcgcaacgttgttgccattgctacaggcatcgtggtgtcacgctcgtcgtttggtatggcttcattcagctccggttcccaacgatcaaggcgagttacatgatcccccatgttgtgcaaaaaagcggttagctccttcggtcctccgatcgttgtcagaagtaagttggccgcagtgttatcactcatggttatggcagcactgcataattctcttactgtcatgccatccgtaagatgcttttctgtgactggtgagtactcaaccaagtcattctgagaatagtgtatgcggcgaccgagttgctcttgcccggcgtcaatacgggataataccgcgccacatagcagaactttaaaagtgctcatcattggaaaacgttcttcggggcgaaaactctcaaggatcttaccgctgttgagatccagttcgatgtaacccactcgtgcacccaactgatcttcagcatcttttactttcaccagcgtttctgggtgagcaaaaacaggaaggcaaaatgccgcaaaaaagggaataagggcgacacggaaatgttgaatactcatactcttcctttttcaatattattgaagcatttatcagggttattgtctcatgagcggatacatatttgaatgtatttagaaaaataaacaaataggggttccgcgcacatttccccgaaaagtgccacctgacgtctaagaaaccattattatcatgacattaacctataaaaataggcgtatcacgaggccctttcgtctcgcgcgtttcggtgatgacggtgaaaacctctgacacatgcagctcccggagacggtcacagcttgtctgtaagcggatgccgggagcagacaagcccgtcagggcgcgtcagcgggtgttggcgggtgtcggggctggcttaactatgcggcatcagagcagattgtactgagagtgcaccataaaattgtaaacgttaatattttgttaaaattcgcgttaaatttttgttaaatcagctcattttttaaccaataggccgaaatcggcaaaatcccttataaatcaaaagaatagcccgagatagggttgagtgttgttccagtttggaacaagagtccactattaaagaacgtggactccaacgtcaaagggcgaaaaaccgtctatcagggcgatggcccactacgtgaaccatcacccaaatcaagttttttggggtcgaggtgccgtaaagcactaaatcggaaccctaaagggagcccccgatttagagcttgacggggaaagccggcgaacgtggcgagaaaggaagggaagaaagcgaaaggagcgggcgctagggcgctggcaagtgtagcggtcacgctgcgcgtaaccaccacacccgccgcgcttaatgcgccgctacagggcgcgtactatggttgctttgacgtatgcggtgtgaaataccgcacagatgcgtaaggagaaaataccgcatcaggcgcccctgcaggcagctgcgcgctcgctcgctcactgaggccgcccgggcaaagcccgggcgtcgggcgacctttggtcgcccggcctcagtgagcgagcgagcgcgcagagagggagtggccaactccatcactaggggttcctacgcgtcgttacataacttacggtaaatggcccgcctggctgaccgcccaacgacccccgcccattgacgtcaataatgacgtatgttcccatagtaacgccaatagggactttccattgacgtcaatgggtggagtatttacggtaaactgcccacttggcagtacatcaagtgtatcatatgccaagtacgccccctattgacgtcaatgacggtaaatggcccgcctggcattatgcccagtacatgaccttatgggactttcctacttggcagtacatctacgtattagtcatcgctattaccatggtcgaggtgagccccacgttctgcttcactctccccatctcccccccctccccacccccaattttgtatttatttattttttaattattttgtgcagcgatgggggcggggggggggggggggcgcgcgccaggcggggcggggcggggcgaggggcggggcggggcgaggcggagaggtgcggcggcagccaatcagagcggcgcgctccgaaagtttccttttatggcgaggcggcggcggcggcggccctataaaaagcgaagcgcgcggcgggcgggagtcgctgcgacgctgccttcgccccgtgccccgctccgccgccgcctcgcgccgcccgccccggctctgactgaccgcgttactcccacaggtgagcgggcgggacggcccttctcctccgggctgtaattagctgagcaagaggtaagggtttaagggatggttggttggtggggtattaatgtttaattacctggagcacctgcctgaaatcactttttttcaggtaccggtcgccaccatggcgagacccctgtgcacattacttctgttgatggctaccctggcaggcgccctcgccagcgagctgacacaggaccctgccgtgtccgtggccctgaagcagaccgtgacaatcacctgcagaggcgattccctgagatcccactacgcctcctggtaccagaagaagcctggccaggcccccgtgctgctgttttacggcaagaataaccgccccagcggcatccccgatagattttccggcagcgcctccggcaacagagccagcctgacaatcaccggcgcccaggccgaggacgaggctgattactactgcagctccagagataagagcggcagcagactgtccgtgtttggcggcggcaccaagctgaccgtgctcggaggaggaggaagcggaggaggaggctcaggcggcggcggctctgaggtgaggctgagagagtccggcggcggcctggtgaagcccggaggatctctgaggctgtcctgctccgcctccggcttcgattttgacaatgcctggatgacctgggtgagacagccccctggcaagggcctggagtgggtgggaaggatcacaggccccggcgagggctggtccgtggattacgccgagtccgtgaagggcaggttcacaatctccagggataacaccaagaacaccctgtacctggagatgaacaacgtgaggacagaggataccggctactacttttgcgccagaacaggcaagtactacgacttttggttcggctacccccctggcgaggagtacttccaggattggggccagggcaccctggtcattgtgtccagcggcggcggcggcagtggcggcggcggaagcggcggcggcggctctggcggcggcggcagcggcggcggcggctccgacatcgtgatgacccagtctcctgatagcctggccgtgagcctgggcgagagagtgacaatgaactgtaagtctagccagagcctgctgtactccaccaaccagaagaattacctggcctggtatcagcagaagcctggccagtccccaaagctgctgatctattgggcatctacaagggagagcggagtgccagacagattcagcggatccggatctggaaccgacttcaccctgacaatctcctctgtgcaggccgaggacgtggccgtgtactattgccagcagtactatagctacaggacattcggcggcggcaccaagctggagatcaagcgcaccgtggccggaggaggaggatctggcggaggagggtccggcggcggcggctcccaggtgcagctgcagcagagcggaccagaggtggtgaagcctggagcctccgtgaagatgtcttgtaaggccagcggctacaccttcacatcctatgtgatccactgggtgaggcagaagccaggacagggactggactggatcggctacatcaacccttataatgatggcaccgactacgatgagaagtttaagggcaaggccaccctgacatccgataccagcacatccaccgcctatatggagctgagctccctgcggtctgaggacacagccgtgtactattgcgccagagagaaggataactacgcaaccggagcatggttcgcatattggggacagggtaccctggtcaccgtgtctagcgagcccaagagctgtgacaagacacacacctgccctccatgtccagcaccagagctgctgggagggccctccgtgttcctgtttccccctaagccaaaggatacactgatgatctccaggacaccagaggtgacctgcgtggtggtggacgtgtctcacgaggatcctgaggtgaagtttaactggtacgtggacggcgtggaggtgcacaatgccaagaccaagcctagggaggagcagtacaattctacatatcgcgtggtgagcgtgctgaccgtgctgcaccaggattggctgaacggcaaggagtataagtgcaaggtgagcaataaggccctgcctgccccaatcgagaagacaatctccaaggcaaagggacagccaagggagcctcaggtgtacaccctgccaccctctcgcgacgagctgacaaagaaccaggtgagcctgacctgtctggtgaagggcttctatcctagcgatattgccgtggagtgggagtccaatggccagccagagaacaattacaagaccacacctccagtgctggactccgatggctctttctttctgtattccaagctgacagtggacaagtctagatggcagcagggcaacgtgttttcttgtagcgtgatgcacgaggccctgcacaatcactacacccagaagtccctgtctctgagccccggcaagggcggaggaggaagcggaggaggcggctctggcggaggaggttccggaggaggcggaagcggcggaggaggctcttacacctccctgatccactccctgatcgaggagtcccagaatcagcaggagaagaatgagcaggagctgctggagctggataagtgggcctccctgtggaattggttctaggtcgacaatcaacctctggattacaaaatttgtgaaagattgactggtattcttaactatgttgctccttttacgctatgtggatacgctgctttaatgcctttgtatcatgctattgcttcccgtatggctttcattttctcctccttgtataaatcctggttgctgtctctttatgaggagttgtggcccgttgtcaggcaacgtggcgtggtgtgcactgtgtttgctgacgcaacccccactggttggggcattgccaccacctgtcagctcctttccgggactttcgctttccccctccctattgccacggcggaactcatcgccgcctgccttgcccgctgctggacaggggctcggctgttgggcactgacaattccgtggtgttgtcggggaagctgacgtcctttccatggctgctcgcctgtgttgccacctggattctgcgcgggacgtccttctgctacgtcccttcggccctcaatccagcggaccttccttcccgcggcctgctgccggctctgcggcctcttccgcgtcttcgccttcgccctcagacgagtcggatctccctttgggccgcctccccgcgaattcgtttatttgtgaaatttgtgatgctattgctttatttgtaaccatctagctttatttgtgaaatttgtgatgctattgctttatttgtaaccattataagctgcaataaacaagttaacaacaacaattgcattcattttatgtttcaggttcagggggagatgtgggaggttttttaaagtttaaacaggaacccctagtgatggagttggccactccctctctgcgcgctcgctcgctcactgaggccgggcgaccaaaggtcgcccgacgcccgggcggcctcagtgagcgagcgagcgcgcagctgcctgcagg

SEQ ID NO: 25 - DNA, 5612 bp, synthetic construct
  misc_feature 1..5612: note = pKL-Kan-Vsvg
  source 1..5612: mol_type = other DNA
ggccgcgttgctggcgtttttccataggctccgcccccctgacgagcatcacaaaaatcgacgctcaagtcagaggtggcgaaacccgacaggactataaagataccaggcgtttccccctggaagctccctcgtgcgctctcctgttccgaccctgccgcttaccggatacctgtccgcctttctcccttcgggaagcgtggcgctttctcatagctcacgctgtaggtatctcagttcggtgtaggtcgttcgctccaagctgggctgtgtgcacgaaccccccgttcagcccgaccgctgcgccttatccggtaactatcgtcttgagtccaacccggtaagacacgacttatcgccactggcagcagccactggtaacaggattagcagagcgaggtatgtaggcggtgctacagagttcttgaagtggtggcctaactacggctacactagaagaacagtatttggtatctgcgctctgctgaagccagttaccttcggaaaaagagttggtagctcttgatccggcaaacaaaccaccgctggtagcggtggtttttttgtttgcaagcagcagattacgcgcagaaaaaaaggatctcaagaagatcctttgatcttttctacggggtctgacgctcagtggaacgaaaactcacgttaagggattttggtcatgaagcgcttttgaagctcggatccgaacaaacgacccaacacccgtgcgttttattctgtctttttattgccgatcccctcagaagaactcgtcaagaaggcgatagaaggcgatgcgctgcgaatcgggagcggcgataccgtaaagcacgaggaagcggtcagcccattcgccgccaagctcttcagcaatatcacgggtagccaacgctatgtcctgatagcggtccgccacacccagccggccacagtcgatgaatccagaaaagcggccattttccaccatgatattcggcaagcaggcatcgccatgggtcacgacgagatcctcgccgtcgggcatgctcgccttgagcctggcgaacagttcggctggcgcgagcccctgatgctcttcgtccagatcatcctgatcgacaagaccggcttccatccgagtacgtgctcgctcgatgcgatgtttcgcttggtggtcgaatgggcaggtagccggatcaagcgtatgcagccgccgcattgcatcagccatgatggatactttctcggcaggagcaaggtgagatgacaggagatcctgccccggcacttcgcccaatagcagccagtcccttcccgcttcagtgacaacgtcgagcacagctgcgcaaggaacgcccgtcgtggccagccacgatagccgcgctgcctcgtcttgcagttcattcagggcaccggacaggtcggtcttgacaaaaagaaccgggcgcccctgcgctgacagccggaacacggcggcatcagagcagccgattgtctgttgtgcccagtcatagccgaatagcctctccacccaagcggccggagaacctgcgtgcaatccatcttgttcaatcatgcgaaacgatcctcatcctgtctcttgatcagagcttgatcccctgcgccatcagatccttggcggcaagaaagccatccagtttactttgcagggcttcccaaccttaccagaggcctgcgccgcggccagctggctagcaattcccgggttaactctagagacattgattattgactagttattaatagtaatcaattacggggtcattagttcatagcccatatatggagttccgcgttacataacttacggtaaatggcccgcctggctgaccgcccaacgacccccgcccattgacgtcaataatgacgtatgttcccatagtaacgccaatagggactttccattgacgtcaatgggtggagtatttacggtaaactgcccacttggcagtacatcaagtgtatcatatgccaagtacgccccctattgacgtcaatgacggtaaatggcccgcctggcattatgcccagtacatgaccttatgggactttcctacttggcagtacatctacgtattagtcatcgctattaccatggtgatgcggttttggcagtacatcaatgggcgtggatagcggtttgactcacggggatttccaagtctccaccccattgacgtcaatgggagtttgttttggcaccaaaatcaacgggactttccaaaatgtcgtaacaactccgccccattgacgcaaatgggcggtaggcgtgtacggtgggaggtctatataagcagagctcgtttagtgaaccgtcagatcgcctggagacgccatccacgctgttttgacctccatagaagacaccgggaccgatccagcctcccctcgaagcttacatgtggtaccgagctcggatcctgagaacttcagggtgagtctatgggacccttgatgttttctttccccttcttttctatggttaagttcatgtcataggaaggggagaagtaacagggtacacatattgaccaaatcagggtaattttgcatttgtaattttaaaaaatgctttcttcttttaatatacttttttgtttatcttatttctaatactttccctaatctctttctttcagggcaataatgatacaatgtatcatgcctctttgcaccattctaaagaataacagtgataatttctgggttaaggcaatagcaatatttctgcatataaatatttctgcatataaattgtaactgatgtaagaggtttcatattgctaatagcagctacaatccagctaccattctgcttttattttatggttgggataaggctggattattctgagtccaagctaggcccttttgctaatcatgttcatacctcttatcttcctcccacagctcctgggcaacgtgctggtctgtgtgctggcccatcactttggcaaagcacgtgagatctgaattctgacactatgaagtgccttttgtacttagcctttttattcattggggtgaattgcaagttcaccatagtttttccacacaaccaaaaaggaaactggaaaaatgttccttctaattaccattattgcccgtcaagctcagatttaaattggcataatgacttaataggcacagccttacaagtcaaaatgcccaagagtcacaaggctattcaagcagacggttggatgtgtcatgcttccaaatgggtcactacttgtgatttccgctggtatggaccgaagtatataacacattccatccgatccttcactccatctgtagaacaatgcaaggaaagcattgaacaaacgaaacaaggaacttggctgaatccaggcttccctcctcaaagttgtggatatgcaactgtgacggatgccgaagcagtgattgtccaggtgactcctcaccatgtgctggttgatgaatacacaggagaatgggttgattcacagttcatcaacggaaaatgcagcaattacatatgccccactgtccataactctacaacctggcattctgactataaggtcaaagggctatgtgattctaacctcatttccatggacatcaccttcttctcagaggacggagagctatcatccctgggaaaggagggcacagggttcagaagtaactactttgcttatgaaactggaggcaaggcctgcaaaatgcaatactgcaagcattggggagtcagactcccatcaggtgtctggttcgagatggctgataaggatctctttgctgcagccagattccctgaatgcccagaagggtcaagtatctctgctccatctcagacctcagtggatgtaagtctaattcaggacgttgagaggatcttggattattccctctgccaagaaacctggagcaaaatcagagcgggtcttccaatctctccagtggatctcagctatcttgctcctaaaaacccaggaaccggtcctgctttcaccataatcaatggtaccctaaaatactttgagaccagatacatcagagtcgatattgctgctccaatcctctcaagaatggtcggaatgatcagtggaactaccacagaaagggaactgtgggatgactgggcaccatatgaagacgtggaaattggacccaatggagttctgaggaccagttcaggatataagtttcctttatacatgattggacatggtatgttggactccgatcttcatcttagctcaaaggctcaggtgttcgaacatcctcacattcaagacgctgcttcgcaacttcctgatgatgagagtttattttttggtgatactgggctatccaaaaatccaatcgagcttgtagaaggttggttcagtagttggaaaagctctattgcctcttttttctttatcatagggttaatcattggactattcttggttctccgagttggtatccatctttgcattaaattaaagcacaccaagaaaagacagatttatacagacatagagatgaaccgacttggaaagtaactcaaatcctgcacaacagattcttcatgtttggaccaaatcaacttgtgataccatgctcaaagaggcctcaattatatttgagtttttaatttttatgaaaaaaaaaaaaaaaaacggaattcaccccaccagtgcaggctgcctatcagaaagtggtggctggtgtggctaatgccctggcccacaagtatcactaagctcgctttcttgctgtccaatttctattaaaggttcctttgttccctaagtccaactactaaactgggggatattatgaagggccttgagcatctggattctgcctaataaaaaacatttattttcattgcaatgatgtatttaaattatttctgaatattttactaaaaagggaatgtgggaggtcagtgcatttaaaacataaagaaatgaagagctagttcaaaccttgggaaaatacactatatcttaaactccatgaaagaaggtgaggctgcaaacagctaatgcacattggcaacagcccctgatgcctatgccttattcatccctcagaaaaggattcaagtagaggcttgatttggaggttaaagttttgctatgctgtattttagtcgaccattacttattgttttagctgtcctcatgaatgtcttttcactacccatttgcttatcctgcatctctcagccttgactccactcagttctcttgcttagagataccacctttcccctgaagtgttccttccatgttttacggcgagatggtttctcctcgcctggccactcagccttagttgtctctgttgtcttatagaggtctacttgaagaaggaaaaacagggggcatggtttgactgtcctgtgagcccttcttccctgcctcccccactcacagtgacccggaatccctcgacatggcagtctagcactagtgcggccgcagatctgcttcctcgctcactgactcgctgcgctcggtcgttcggctgcggcgagcggtatcagctcactcaaaggcggtaatacggttatccacagaatcaggggataacgcaggaaagaacatgtgagcaaaaggccagcaaaaggccaggaaccgtaaaaa

SEQ ID NO: 26 - DNA, 3387 bp, synthetic construct
  misc_feature 1..3387: note = pKL-Kan-Rev
  source 1..3387: mol_type = other DNA
ggccgcgttgctggcgtttttccataggctccgcccccctgacgagcatcacaaaaatcgacgctcaagtcagaggtggcgaaacccgacaggactataaagataccaggcgtttccccctggaagctccctcgtgcgctctcctgttccgaccctgccgcttaccggatacctgtccgcctttctcccttcgggaagcgtggcgctttctcatagctcacgctgtaggtatctcagttcggtgtaggtcgttcgctccaagctgggctgtgtgcacgaaccccccgttcagcccgaccgctgcgccttatccggtaactatcgtcttgagtccaacccggtaagacacgacttatcgccactggcagcagccactggtaacaggattagcagagcgaggtatgtaggcggtgctacagagttcttgaagtggtggcctaactacggctacactagaagaacagtatttggtatctgcgctctgctgaagccagttaccttcggaaaaagagttggtagctcttgatccggcaaacaaaccaccgctggtagcggtggtttttttgtttgcaagcagcagattacgcgcagaaaaaaaggatctcaagaagatcctttgatcttttctacggggtctgacgctcagtggaacgaaaactcacgttaagggattttggtcatgaagcgcttttgaagctcggatccgaacaaacgacccaacacccgtgcgttttattctgtctttttattgccgatcccctcagaagaactcgtcaagaaggcgatagaaggcgatgcgctgcgaatcgggagcggcgataccgtaaagcacgaggaagcggtcagcccattcgccgccaagctcttcagcaatatcacgggtagccaacgctatgtcctgatagcggtccgccacacccagccggccacagtcgatgaatccagaaaagcggccattttccaccatgatattcggcaagcaggcatcgccatgggtcacgacgagatcctcgccgtcgggcatgctcgccttgagcctggcgaacagttcggctggcgcgagcccctgatgctcttcgtccagatcatcctgatcgacaagaccggcttccatccgagtacgtgctcgctcgatgcgatgtttcgcttggtggtcgaatgggcaggtagccggatcaagcgtatgcagccgccgcattgcatcagccatgatggatactttctcggcaggagcaaggtgagatgacaggagatcctgccccggcacttcgcccaatagcagccagtcccttcccgcttcagtgacaacgtcgagcacagctgcgcaaggaacgcccgtcgtggccagccacgatagccgcgctgcctcgtcttgcagttcattcagggcaccggacaggtcggtcttgacaaaaagaaccgggcgcccctgcgctgacagccggaacacggcggcatcagagcagccgattgtctgttgtgcccagtcatagccgaatagcctctccacccaagcggccggagaacctgcgtgcaatccatcttgttcaatcatgcgaaacgatcctcatcctgtctcttgatcagagcttgatcccctgcgccatcagatccttggcggcaagaaagccatccagtttactttgcagggcttcccaaccttaccagaggcctgcgccgcggccagctggctagcaattcccgggttaactctagagaatgtagtcttatgcaatactcttgtagtcttgcaacatggtaacgatgagttagcaacatgccttacaaggagagaaaaagcaccgtgcatgccgattggtggaagtaaggtggtacgatcgtgccttattaggaaggcaacagacgggtctgacatggattggacgaaccactgaattccgcattgcagagatattgtatttaagtgcctagctcgatacaataaacgccatttgaccattcaccacattggtgtgcacctccaagctcgagctcgtttagtgaaccgtcagatcgcctggagacgccatccacgctgttttgacctccatagaagacaccgggaccgatccagcctcccctcgaagctagtcgattaggcatctcctatggcaggaagaagcggagacagcgacgaagacctcctcaaggcagtcagactcatcaagtttctctatcaaagcaacccacctcccaatcccgaggggacccgacaggcccgaaggaatagaagaagaaggtggagagagagacagagacagatccattcgattagtgaacggatccttagcacttatctgggacgatctgcggagcctgtgcctcttcagctaccaccgcttgagagacttactcttgattgtaacgaggattgtggaacttctgggacgcagggggtgggaagccctcaaatattggtggaatctcctacaatattggagtcaggagctaaagaatagtgctgttagcttgctcaatgccacagctatagcagtagctgaggggacagatagggttatagaagtagtacaagaagcttggcactggccgtcgttttacaacgtcgtgatctgagcctgggagatctctggctaactagggaacccactgcttaagcctcaataaagcttgccttgagtgcttcaagtagtgtgtgcccgtctgttgtgtgactctggtaactagagatcaggaaaaccctggcgttacccaacttaatcgccttgcagcacatccccctttcgccagctggcgtaatagcgaagaggcccgcaccgatcgcccttcccaacagttgcgcagcctgaatggcgaatggcgcctgatgcggtattttctccttacgcatctgtgcggtatttcacaccgcatacgtcaaagcaaccatagtgtcgaccattacttattgttttagctgtcctcatgaatgtcttttcactacccatttgcttatcctgcatctctcagccttgactccactcagttctcttgcttagagataccacctttcccctgaagtgttccttccatgttttacggcgagatggtttctcctcgcctggccactcagccttagttgtctctgttgtcttatagaggtctacttgaagaaggaaaaacagggggcatggtttgactgtcctgtgagcccttcttccctgcctcccccactcacagtgacccggaatccctcgacatggcagtctagcactagtgcggccgcagatctgcttcctcgctcactgactcgctgcgctcggtcgttcggctgcggcgagcggtatcagctcactcaaaggcggtaatacggttatccacagaatcaggggataacgcaggaaagaacatgtgagcaaaaggccagcaaaaggccaggaaccgtaaaaa

SEQ ID NO: 27 - DNA, 9171 bp, synthetic construct
  misc_feature 1..9171: note = pKL-Kan-GagPol
  source 1..9171: mol_type = other DNA
ggccgcgttgctggcgtttttccataggctccgcccccctgacgagcatcacaaaaatcgacgctcaagtcagaggtggcgaaacccgacaggactataaagataccaggcgtttccccctggaagctccctcgtgcgctctcctgttccgaccctgccgcttaccggatacctgtccgcctttctcccttcgggaagcgtggcgctttctcatagctcacgctgtaggtatctcagttcggtgtaggtcgttcgctccaagctgggctgtgtgcacgaaccccccgttcagcccgaccgctgcgccttatccggtaactatcgtcttgagtccaacccggtaagacacgacttatcgccactggcagcagccactggtaacaggattagcagagcgaggtatgtaggcggtgctacagagttcttgaagtggtggcctaactacggctacactagaagaacagtatttggtatctgcgctctgctgaagccagttaccttcggaaaaagagttggtagctcttgatccggcaaacaaaccaccgctggtagcggtggtttttttgtttgcaagcagcagattacgcgcagaaaaaaaggatctcaagaagatcctttgatcttttctacggggtctgacgctcagtggaacgaaaactcacgttaagggattttggtcatgaagcgcttttgaagctcggatccgaacaaacgacccaacacccgtgcgttttattctgtctttttattgccgatcccctcagaagaactcgtcaagaaggcgatagaaggcgatgcgctgcgaatcgggagcggcgataccgtaaagcacgaggaagcggtcagcccattcgccgccaagctcttcagcaatatcacgggtagccaacgctatgtcctgatagcggtccgccacacccagccggccacagtcgatgaatccagaaaagcggccattttccaccatgatattcggcaagcaggcatcgccatgggtcacgacgagatcctcgccgtcgggcatgctcgccttgagcctggcgaacagttcggctggcgcgagcccctgatgctcttcgtccagatcatcctgatcgacaagaccggcttccatccgagtacgtgctcgctcgatgcgatgtttcgcttggtggtcgaatgggcaggtagccggatcaagcgtatgcagccgccgcattgcatcagccatgatggatactttctcggcaggagcaaggtgagatgacaggagatcctgccccggcacttcgcccaatagcagccagtcccttcccgcttcagtgacaacgtcgagcacagctgcgcaaggaacgcccgtcgtggccagccacgatagccgcgctgcctcgtcttgcagttcattcagggcaccggacaggtcggtcttgacaaaaagaaccgggcgcccctgcgctgacagccggaacacggcggcatcagagcagccgattgtctgttgtgcccagtcatagccgaatagcctctccacccaagcggccggagaacctgcgtgcaatccatcttgttcaatcatgcgaaacgatcctcatcctgtctcttgatcagagcttgatcccctgcgccatcagatccttggcggcaagaaagccatccagtttactttgcagggcttcccaaccttaccagaggcctgcgccgcggccagctggctagcaattcccgggttaactctagagacattgattattgactagttattaatagtaatcaattacggggtcattagttcatagcccatatatggagttccgcgttacataacttacggtaaatggcccgcctggctgaccgcccaacgacccccgcccattgacgtcaataatgacgtatgttcccatagtaacgccaatagggactttccattgacgtcaatgggtggagtatttacggtaaactgcccacttggcagtacatcaagtgtatcatatgccaagtacgccccctattgacgtcaatgacggtaaatggcccgcctggcattatgcccagtacatgaccttatgggactttcctacttggcagtacatctacgtattagtcatcgctattaccatggtgatgcggttttggcagtacatcaatgggcgtggatagcggtttgactcacggggatttccaagtctccaccccattgacgtcaatgggagtttgttttggcaccaaaatcaacgggactttccaaaatgtcgtaacaactccgccccattgacgcaaatgggcggtaggcgtgtacggtgggaggtctatataagcagagctcgtttagtgaaccgtcagatcgcctggagacgccatccacgctgttttgacctccatagaagacaccgggaccgatccagcctcccctcgaagcttacatgtggtaccgagctcggatcctgagaacttcagggtgagtctatgggacccttgatgttttctttccccttcttttctatggttaagttcatgtcataggaaggggagaagtaacagggtacacatattgaccaaatcagggtaattttgcatttgtaattttaaaaaatgctttcttcttttaatatacttttttgtttatcttatttctaatactttccctaatctctttctttcagggcaataatgatacaatgtatcatgcctctttgcaccattctaaagaataacagtgataatttctgggttaaggcaatagcaatatttctgcatataaatatttctgcatataaattgtaactgatgtaagaggtttcatattgctaatagcagctacaatccagctaccattctgcttttattttatggttgggataaggctggattattctgagtccaagctaggcccttttgctaatcatgttcatacctcttatcttcctcccacagctcctgggcaacgtgctggtctgtgtgctggcccatcactttggcaaagcacgtgagatctgaattcgagatctgccgccgccatgggtgcgagagcgtcagtattaagcgggggagaattagatcgatgggaaaaaattcggttaaggccagggggaaagaaaaaatataaattaaaacatatagtatgggcaagcagggagctagaacgattcgcagttaatcctggcctgttagaaacatcagaaggctgtagacaaatactgggacagctacaaccatcccttcagacaggatcagaagaacttagatcattatataatacagtagcaaccctctattgtgtgcatcaaaggatagagataaaagacaccaaggaagctttagacaagatagaggaagagcaaaacaaaagtaagaaaaaagcacagcaagcagcagctgacacaggacacagcaatcaggtcagccaaaattaccctatagtgcagaacatccaggggcaaatggtacatcaggccatatcacctagaactttaaatgcatgggtaaaagtagtagaagagaaggctttcagcccagaagtgatacccatgttttcagcattatcagaaggagccaccccacaagatttaaacaccatgctaaacacagtggggggacatcaagcagccatgcaaatgttaaaagagaccatcaatgaggaagctgcagaatgggatagagtgcatccagtgcatgcagggcctattgcaccaggccagatgagagaaccaaggggatcagacatcgctggaactactagtacccttcaggaacaaataggatggatgacacataatccacctatcccagtaggagaaatctataaaagatggataatcctgggattaaataaaatagtaagaatgtatagccctaccagcattctggacataagacaaggaccaaaggaaccctttagagactatgtagaccgattctataaaactctaagagccgagcaagcttcacaagaggtaaaaaattggatgacagaaaccttgttggtccaaaatgcgaacccagattgtaagactattttaaaagcattgggaccaggagcgacactagaagaaatgatgacagcatgtcagggagtggggggacccggccataaagcaagagttttggctgaagcaatgagccaagtaacaaatccagctaccataatgatacagaaaggcaattttaggaaccaaagaaagactgttaagtgtttcaattgtggcaaagaagggcacatagccaaaaattgcagggcccctaggaaaaagggctgttggaaatgtggaaaggaaggacaccaaatgaaagattgtactgagagacaggctaattttttagggaagatctggccttcccacaagggaaggccagggaattttcttcagagcagaccagagccaacagccccaccagaagagagcttcaggtttggggaagagacaacaactccctctcagaagcaggagccgatagacaaggaactgtatcctttagcttccctcagatcactctttggcagcgacccctcgtcacaataaagataggggggcaattaaaggaagctctattagatactggtgctgacgacacagtattagaagaaatgaatttgccaggaagatggaaaccaaaaatgatagggggaattggaggttttatcaaagtaagacagtatgatcagatactcatagaaatctgcggacataaagctataggtacagtattagtaggacctacacctgtcaacataattggaagaaatctgttgactcagattggctgcactttaaattttcccattagtcctattgagactgtaccagtaaaattaaagccaggaatggatggcccaaaagttaaacaatggccattgacagaagaaaaaataaaagcattagtagaaatttgtacagaaatggaaaaggaaggaaaaatttcaaaaattgggcctgaaaatccatacaatactccagtatttgccataaagaaaaaagacagtactaaatggagaaaattagtagatttcagagaacttaataagagaactcaagatttctgggaagttcaattaggaataccacatcctgcagggttaaaacagaaaaaatcagtaacagtactggatgtgggcgatgcatatttttcagttcccttagataaagacttcaggaagtatactgcatttaccatacctagtataaacaatgagacaccagggattagatatcagtacaatgtgcttccacagggatggaaaggatcaccagcaatattccagtgtagcatgacaaaaatcttagagccttttagaaaacaaaatccagacatagtcatctatcaatacatggatgatttgtatgtaggatctgacttagaaatagggcagcatagaacaaaaatagaggaactgagacaacatctgttgaggtggggatttaccacaccagacaaaaaacatcagaaagaacctccattcctttggatgggttatgaactccatcctgataaatggacagtacagcctatagtgctgccagaaaaggacagctggactgtcaatgacatacagaaattagtgggaaaattgaattgggcaagtcagatttatgcagggattaaagtaaggcaattatgtaaacttcttaggggaaccaaagcactaacagaagtagtaccactaacagaagaagcagagctagaactggcagaaaacagggagattctaaaagaaccggtacatggagtgtattatgacccatcaaaagacttaatagcagaaatacagaagcaggggcaaggccaatggacatatcaaatttatcaagagccatttaaaaatctgaaaacaggaaagtatgcaagaatgaagggtgcccacactaatgatgtgaaacaattaacagaggcagtacaaaaaatagccacagaaagcatagtaatatggggaaagactcctaaatttaaattacccatacaaaaggaaacatgggaagcatggtggacagagtattggcaagccacctggattcctgagtgggagtttgtcaatacccctcccttagtgaagttatggtaccagttagagaaagaacccataataggagcagaaactttctatgtagatggggcagccaatagggaaactaaattaggaaaagcaggatatgtaactgacagaggaagacaaaaagttgtccccctaacggacacaacaaatcagaagactgagttacaagcaattcatctagctttgcaggattcgggattagaagtaaacatagtgacagactcacaatatgcattgggaatcattcaagcacaaccagataagagtgaatcagagttagtcagtcaaataatagagcagttaataaaaaaggaaaaagtctacctggcatgggtaccagcacacaaaggaattggaggaaatgaacaagtagataaattggtcagtgctggaatcaggaaagtactatttttagatggaatagataaggcccaagaagaacatgagaaatatcacagtaattggagagcaatggctagtgattttaacctaccacctgtagtagcaaaagaaatagtagccagctgtgataaatgtcagctaaaaggggaagccatgcatggacaagtagactgtagcccaggaatatggcagctagattgtacacatttagaaggaaaagttatcttggtagcagttcatgtagccagtggatatatagaagcagaagtaattccagcagagacagggcaagaaacagcatacttcctcttaaaattagcaggaagatggccagtaaaaacagtacatacagacaatggcagcaatttcaccagtactacagttaaggccgcctgttggtgggcggggatcaagcaggaatttggcattccctacaatccgcagtcacaaggagtaatagaatctatgaataaagaattaaagaaaattataggacaggtaagagatcaggctgaacatcttaaaacagcagtacaaatggcagtattcatccacaattttaaaagaaaaggggggattggggggtacagtgcaggggaaagaatagtagacataatagcaacagacatacaaactaaagaattacaaaaacaaattacaaaaattcaaaattttcgggtttattacagggacagcagagatccagtttggaaaggaccagcaaagctcctctggaaaggtgaaggggcagtagtaatacaagataatagtgacataaaagtagtgccaagaagaaaagcaaagatcatcagggattatggaaaacagatggcaggtgatgattgtgtggcaagtagacaggatgaggattaacacatggaattccggagcggccgcaggagctttgttccttgggttcttgggagcagcaggaagcactatgggcgcagcgtcaatgacgctgacggtacaggccagacaattattgtctggtatagtgcagcagcagaacaatttgctgagggctattgaggcgcaacagcatctgttgcaactcacagtctggggcatcaagcagctccaggcaagaatcctggctgtggaaagatacctaaaggatcaacagctcctggggatttggggttgctctggaaaactcatttgcaccactgctgtgccttggaatgctagttggagtaataaatctctggaacagatttggaatcacacgacctggatggagtgggacagagaaattaacaattacacaagcttccgcggaattcaccccaccagtgcaggctgcctatcagaaagtggtggctggtgtggctaatgccctggcccacaagtatcactaagctcgctttcttgctgtccaatttctattaaaggttcctttgttccctaagtccaactactaaactgggggatattatgaagggccttgagcatctggattctgcctaataaaaaacatttattttcattgcaatgatgtatttaaattatttctgaatattttactaaaaagggaatgtgggaggtcagtgcatttaaaacataaagaaatgaagagctagttcaaaccttgggaaaatacactatatcttaaactccatgaaagaaggtgaggctgcaaacagctaatgcacattggcaacagcccctgatgcctatgccttattcatccctcagaaaaggattcaagtagaggcttgatttggaggttaaagttttgctatgctgtattttacattacttattgttttagctgtcctcatgaatgtcttttcactacccatttgcttatcctgcatctctcagccttgactccactcagttctcttgcttagagataccacctttcccctgaagtgttccttccatgttttacggcgagatggtttctcctcgcctggccactcagccttagttgtctctgttgtcttatagaggtctacttgaagaaggaaaaacagggggcatggtttgactgtcctgtgagcccttcttccctgcctcccccactcacagtgacccggaatccctcgacatggcagtctagcactagtgcggccgcagatctgcttcctcgctcactgactcgctgcgctcggtcgttcggctgcggcgagcggtatcagctcactcaaaggcggtaatacggttatccacagaatcaggggataacgcaggaaagaacatgtgagcaaaaggccagcaaaaggccaggaaccgtaaaaagtcgaccattacttattgttttagctgtcctcatgaatgtcttttcactacccatttgcttatcctgcatctctcagccttgactccactcagttctcttgcttagagataccacctttcccctgaagtgttccttccatgttttacggcgagatggtttctcctcgcctggccactcagccttagttgtctctgttgtcttatagaggtctacttgaagaaggaaaaacagggggcatggtttgactgtcctgtgagcccttcttccctgcctcccccactcacagtgacccggaatccctcgacatggcagtctagcactagtgcggccgcagatctgcttcctcgctcactgactcgctgcgctcggtcgttcggctgcggcgagcggtatcagctcactcaaaggcggtaatacggttatccacagaatcaggggataacgcaggaaagaacatgtgagcaaaaggccagcaaaaggccaggaaccgtaaaaa

SEQ ID NO: 28 - DNA, 7336 bp, synthetic construct
  source 1..7336: mol_type = other DNA; note = AAV2/8
atgccggggttttacgagattgtgattaaggtccccagcgaccttgacgagcatctgcccggcatttctgacagctttgtgaactgggtggccgagaaggaatgggagttgccgccagattctgacatggatctgaatctgattgagcaggcacccctgaccgtggccgagaagctgcagcgcgactttctgacggaatggcgccgtgtgagtaaggccccggaggctcttttctttgtgcaatttgagaagggagagagctacttccacatgcacgtgctcgtggaaaccaccggggtgaaatccatggttttgggacgtttcctgagtcagattcgcgaaaaactgattcagagaatttaccgcgggatcgagccgactttgccaaactggttcgcggtcacaaagaccagaaatggcgccggaggcgggaacaaggtggtggatgagtgctacatccccaattacttgctccccaaaacccagcctgagctccagtgggcgtggactaatatggaacagtatttaagcgcctgtttgaatctcacggagcgtaaacggttggtggcgcagcatctgacgcacgtgtcgcagacgcaggagcagaacaaagagaatcagaatcccaattctgatgcgccggtgatcagatcaaaaacttcagccaggtacatggagctggtcgggtggctcgtggacaaggggattacctcggagaagcagtggatccaggaggaccaggcctcatacatctccttcaatgcggcctccaactcgcggtcccaaatcaaggctgccttggacaatgcgggaaagattatgagcctgactaaaaccgcccccgactacctggtgggccagcagcccgtggaggacatttccagcaatcggatttataaaattttggaactaaacgggtacgatccccaatatgcggcttccgtctttctgggatgggccacgaaaaagttcggcaagaggaacaccatctggctgtttgggcctgcaactaccgggaagaccaacatcgcggaggccatagcccacactgtgcccttctacgggtgcgtaaactggaccaatgagaactttcccttcaacgactgtgtcgacaagatggtgatctggtgggaggaggggaagatgaccgccaaggtcgtggagtcggccaaagccattctcggaggaagcaaggtgcgcgtggaccagaaatgcaagtcctcggcccagatagacccgactcccgtgatcgtcacctccaacaccaacatgtgcgccgtgattgacgggaactcaacgaccttcgaacaccagcagccgttgcaagaccggatgttcaaatttgaactcacccgccgtctggatcatgactttgggaaggtcaccaagcaggaagtcaaagactttttccggtgggcaaaggatcacgtggttgaggtggagcatgaattctacgtcaaaaagggtggagccaagaaaagacccgcccccagtgacgcagatataagtgagcccaaacgggtgcgcgagtcagttgcgcagccatcgacgtcagacgcggaagcttcgatcaactacgcagacaggtaccaaaacaaatgttctcgtcacgtgggcatgaatctgatgctgtttccctgcagacaatgcgagagaatgaatcagaattcaaatatctgcttcactcacggacagaaagactgtttagagtgctttcccgtgtcagaatctcaacccgtttctgtcgtcaaaaaggcgtatcagaaactgtgctacattcatcatatcatgggaaaggtgccagacgcttgcactgcctgcgatctggtcaatgtggatttggatgactgcatctttgaacaataaatgatttaaatcaggtatggctgccgatggttatcttccagattggctcgaggacaacctctctgagggcattcgcgagtggtgggcgctgaaacctggagccccgaagcccaaagccaaccagcaaaagcaggacgacggccggggtctggtgcttcctggctacaagtacctcggacccttcaacggactcgacaagggggagcccgtcaacgcggcggacgcagcggccctcgagcacgacaaggcctacgaccagcagctgcaggcgggtgacaatccgtacctgcggtataaccacgccgacgccgagtttcaggagcgtctgcaagaagatacgtcttttgggggcaacctcgggcgagcagtcttccaggccaagaagcgggttctcgaacctctcggtctggttgaggaaggcgctaagacggctcctggaaagaagagaccggtagagccatcaccccagcgttctccagactcctctacgggcatcggcaagaaaggccaacagcccgccagaaaaagactcaattttggtcagactggcgactcagagtcagttccagaccctcaacctctcggagaacctccagcagcgccctctggtgtgggacctaatacaatggctgcaggcggtggcgcaccaatggcagacaataacgaaggcgccgacggagtgggtagttcctcgggaaattggcattgcgattccacatggctgggcgacagagtcatcaccaccagcacccgaacctgggccctgcccacctacaacaaccacctctacaagcaaatctccaacgggacatcgggaggagccaccaacgacaacacctacttcggctacagcaccccctgggggtattttgactttaacagattccactgccacttttcaccacgtgactggcagcgactcatcaacaacaactggggattccggcccaagagactcagcttcaagctcttcaacatccaggtcaaggaggtcacgcagaatgaaggcaccaagaccatcgccaataacctcaccagcaccatccaggtgtttacggactcggagtaccagctgccgtacgttctcggctctgcccaccagggctgcctgcctccgttcccggcggacgtgttcatgattccccagtacggctacctaacactcaacaacggtagtcaggccgtgggacgctcctccttctactgcctggaatactttccttcgcagatgctgagaaccggcaacaacttccagtttacttacaccttcgaggacgtgcctttccacagcagctacgcccacagccagagcttggaccggctgatgaatcctctgattgaccagtacctgtactacttgtctcggactcaaacaacaggaggcacggcaaatacgcagactctgggcttcagccaaggtgggcctaatacaatggccaatcaggcaaagaactggctgccaggaccctgttaccgccaacaacgcgtctcaacgacaaccgggcaaaacaacaatagcaactttgcctggactgctgggaccaaataccatctgaatggaagaaattcattggctaatcctggcatcgctatggcaacacacaaagacgacgaggagcgtttttttcccagtaacgggatcctgatttttggcaaacaaaatgctgccagagacaatgcggattacagcgatgtcatgctcaccagcgaggaagaaatcaaaaccactaaccctgtggctacagaggaatacggtatcgtggcagataacttgcagcagcaaaacacggctcctcaaattggaactgtcaacagccagggggccttacccggtatggtctggcagaaccgggacgtgtacctgcagggtcccatctgggccaagattcctcacacggacggcaacttccacccgtctccgctgatgggcggctttggcctgaaacatcctccgcctcagatcctgatcaagaacacgcctgtacctgcggatcctccgaccaccttcaaccagtcaaagctgaactctttcatcacgcaatacagcaccggacaggtcagcgtggaaattgaatgggagctgcagaaggaaaacagcaagcgctggaaccccgagatccagtacacctccaactactacaaatctacaagtgtggactttgctgttaatacagaaggcgtgtactctgaaccccgccccattggcacccgttacctcacccgtaatctgtaattgcctgttaatcaataaaccggttgattcgtttcagttgaactttggtctctgcgaagggcgaattcgtttaaacctgcaggactagaggtcctgtattagaggtcacgtgagtgttttgcgacattttgcgacaccatgtggtcacgctgggtatttaagcccgagtgagcacgcagggtctccattttgaagcgggaggtttgaacgcgcagccgccaagccgaattctgcagatatccatcacactggcggccgctcgactagagcggccgccaccgcggtggagctccagcttttgttccctttagtgagggttaattgcgcgcttggcgtaatcatggtcatagctgtttcctgtgtgaaattgttatccgctcacaattccacacaacatacgagccggaagcataaagtgtaaagcctggggtgcctaatgagtgagctaactcacattaattgcgttgcgctcactgcccgctttccagtcgggaaacctgtcgtgccagctgcattaatgaatcggccaacgcgcggggagaggcggtttgcgtattgggcgctcttccgcttcctcgctcactgactcgctgcgctcggtcgttcggctgcggcgagcggtatcagctcactcaaaggcggtaatacggttatccacagaatcaggggataacgcaggaaagaacatgtgagcaaaaggccagcaaaaggccaggaaccgtaaaaaggccgcgttgctggcgtttttccataggctccgcccccctgacgagcatcacaaaaatcgacgctcaagtcagaggtggcgaaacccgacaggactataaagataccaggcgtttccccctggaagctccctcgtgcgctctcctgttccgaccctgccgcttaccggatacctgtccgcctttctcccttcgggaagcgtggcgctttctcatagctcacgctgtaggtatctcagttcggtgtaggtcgttcgctccaagctgggctgtgtgcacgaaccccccgttcagcccgaccgctgcgccttatccggtaactatcgtcttgagtccaacccggtaagacacgacttatcgccactggcagcagccactggtaacaggattagcagagcgaggtatgtaggcggtgctacagagttcttgaagtggtggcctaactacggctacactagaagaacagtatttggtatctgcgctctgctgaagccagttaccttcggaaaaagagttggtagctcttgatccggcaaacaaaccaccgctggtagcggtggtttttttgtttgcaagcagcagattacgcgcagaaaaaaaggatctcaagaagatcctttgatcttttctacggggtctgacgctcagtggaacgaaaactcacgttaagggattttggtcatgagattatcaaaaaggatcttcacctagatccttttaaattaaaaatgaagttttaaatcaatctaaagtatatatgagtaaacttggtctgacagttaccaatgcttaatcagtgaggcacctatctcagcgatctgtctatttcgttcatccatagttgcctgactccccgtcgtgtagataactacgatacgggagggcttaccatctggccccagtgctgcaatgataccgcgagacccacgctcaccggctccagatttatcagcaataaaccagccagccggaagggccgagcgcagaagtggtcctgcaactttatccgcctccatccagtctattaattgttgccgggaagctagagtaagtagttcgccagttaatagtttgcgcaacgttgttgccattgctacaggcatcgtggtgtcacgctcgtcgtttggtatggcttcattcagctccggttcccaacgatcaaggcgagttacatgatcccccatgttgtgcaaaaaagcggttagctccttcggtcctccgatcgttgtcagaagtaagttggccgcagtgttatcactcatggttatggcagcactgcataattctcttactgtcatgccatccgtaagatgcttttctgtgactggtgagtactcaaccaagtcattctgagaatagtgtatgcggcgaccgagttgctcttgcccggcgtcaatacgggataataccgcgccacatagcagaactttaaaagtgctcatcattggaaaacgttcttcggggcgaaaactctcaaggatcttaccgctgttgagatccagttcgatgtaacccactcgtgcacccaactgatcttcagcatcttttactttcaccagcgtttctgggtgagcaaaaacaggaaggcaaaatgccgcaaaaaagggaataagggcgacacggaaatgttgaatactcatactcttcctttttcaatattattgaagcatttatcagggttattgtctcatgagcggatacatatttgaatgtatttagaaaaataaacaaataggggttccgcgcacatttccccgaaaagtgccacctaaattgtaagcgttaatattttgttaaaattcgcgttaaatttttgttaaatcagctcattttttaaccaataggccgaaatcggcaaaatcccttataaatcaaaagaatagaccgagatagggttgagtgttgttccagtttggaacaagagtccactattaaagaacgtggactccaacgtcaaagggcgaaaaaccgtctatcagggcgatggcccactacgtgaaccatcaccctaatcaagttttttggggtcgaggtgccgtaaagcactaaatcggaaccctaaagggagcccccgatttagagcttgacggggaaagccggcgaacgtggcgagaaaggaagggaagaaagcgaaaggagcgggcgctagggcgctggcaagtgtagcggtcacgctgcgcgtaaccaccacacccgccgcgcttaatgcgccgctacagggcgcgtcccattcgccattcaggctgcgcaactgttgggaagggcgatcggtgcgggcctcttcgctattacgccagctggcgaaagggggatgtgctgcaaggcgattaagttgggtaacgccagggttttcccagtcacgacgttgtaaaacgacggccagtgagcgcgcgtaatacgactcactatagggcgaattgggtaccgggccccccctcgatcgaggtcgacggtatcgggggagctcgcagggtctccattttgaagcgggaggtttgaacgcgcagccgcc

SEQ ID NO: 29 - DNA, 11635 bp, synthetic construct
  source 1..11635: mol_type = other DNA; note = pHelper
ggtacccaactccatgcttaacagtccccaggtacagcccaccctgcgtcgcaaccaggaacagctctacagcttcctggagcgccactcgccctacttccgcagccacagtgcgcagattaggagcgccacttctttttgtcacttgaaaaacatgtaaaaataatgtactaggagacactttcaataaaggcaaatgtttttatttgtacactctcgggtgattatttaccccccacccttgccgtctgcgccgtttaaaaatcaaaggggttctgccgcgcatcgctatgcgccactggcagggacacgttgcgatactggtgtttagtgctccacttaaactcaggcacaaccatccgcggcagctcggtgaagttttcactccacaggctgcgcaccatcaccaacgcgtttagcaggtcgggcgccgatatcttgaagtcgcagttggggcctccgccctgcgcgcgcgagttgcgatacacagggttgcagcactggaacactatcagcgccgggtggtgcacgctggccagcacgctcttgtcggagatcagatccgcgtccaggtcctccgcgttgctcagggcgaacggagtcaactttggtagctgccttcccaaaaagggtgcatgcccaggctttgagttgcactcgcaccgtagtggcatcagaaggtgaccgtgcccggtctgggcgttaggatacagcgcctgcatgaaagccttgatctgcttaaaagccacctgagcctttgcgccttcagagaagaacatgccgcaagacttgccggaaaactgattggccggacaggccgcgtcatgcacgcagcaccttgcgtcggtgttggagatctgcaccacatttcggccccaccggttcttcacgatcttggccttgctagactgctccttcagcgcgcgctgcccgttttcgctcgtcacatccatttcaatcacgtgctccttatttatcataatgctcccgtgtagacacttaagctcgccttcgatctcagcgcagcggtgcagccacaacgcgcagcccgtgggctcgtggtgcttgtaggttacctctgcaaacgactgcaggtacgcctgcaggaatcgccccatcatcgtcacaaaggtcttgttgctggtgaaggtcagctgcaacccgcggtgctcctcgtttagccaggtcttgcatacggccgccagagcttccacttggtcaggcagtagcttgaagtttgcctttagatcgttatccacgtggtacttgtccatcaacgcgcgcgcagcctccatgcccttctcccacgcagacacgatcggcaggctcagcgggtttatcaccgtgctttcactttccgcttcactggactcttccttttcctcttgcgtccgcataccccgcgccactgggtcgtcttcattcagccgccgcaccgtgcgcttacctcccttgccgtgcttgattagcaccggtgggttgctgaaacccaccatttgtagcgccacatcttctctttcttcctcgctgtccacgatcacctctggggatggcgggcgctcgggcttgggagaggggcgcttctttttctttttggacgcaatggccaaatccgccgtcgaggtcgatggccgcgggctgggtgtgcgcggcaccagcgcatcttgtgacgagtcttcttcgtcctcggactcgagacgccgcctcagccgcttttttgggggcgcgcggggaggcggcggcgacggcgacggggacgacacgtcctccatggttggtggacgtcgcgccgcaccgcgtccgcgctcgggggtggtttcgcgctgctcctcttcccgactggccatttccttctcctataggcagaaaaagatcatggagtcagtcgagaaggaggacagcctaaccgccccctttgagttcgccaccaccgcctccaccgatgccgccaacgcgcctaccaccttccccgtcgaggcacccccgcttgaggaggaggaagtgattatcgagcaggacccaggttttgtaagcgaagacgacgaggatcgctcagtaccaacagaggataaaaagcaagaccaggacgacgcagaggcaaacgaggaacaagtcgggcggggggaccaaaggcatggcgactacctagatgtgggagacgacgtgctgttgaagcatctgcagcgccagtgcgccattatctgcgacgcgttgcaagagcgcagcgatgtgcccctcgccatagcggatgtcagccttgcctacgaacgccacctgttctcaccgcgcgtaccccccaaacgccaagaaaacggcacatgcgagcccaacccgcgcctcaacttctaccccgtatttgccgtgccagaggtgcttgccacctatcacatctttttccaaaactgcaagatacccctatcctgccgtgccaaccgcagccgagcggacaagcagctggccttgcggcagggcgctgtcatacctgatatcgcctcgctcgacgaagtgccaaaaatctttgagggtcttggacgcgacgagaaacgcgcggcaaacgctctgcaacaagaaaacagcgaaaatgaaagtcactgtggagtgctggtggaacttgagggtgacaacgcgcgcctagccgtgctgaaacgcagcatcgaggtcacccactttgcctacccggcacttaacctaccccccaaggttatgagcacagtcatgagcgagctgatcgtgcgccgtgcacgacccctggagagggatgcaaacttgcaagaacaaaccgaggagggcctacccgcagttggcgatgagcagctggcgcgctggcttgagacgcgcgagcctgccgacttggaggagcgacgcaagctaatgatggccgcagtgcttgttaccgtggagcttgagtgcatgcagcggttctttgctgacccggagatgcagcgcaagctagaggaaacgttgcactacacctttcgccagggctacgtgcgccaggcctgcaaaatttccaacgtggagctctgcaacctggtctcctaccttggaattttgcacgaaaaccgcctcgggcaaaacgtgcttcattccacgctcaagggcgaggcgcgccgcgactacgtccgcgactgcgtttacttatttctgtgctacacctggcaaacggccatgggcgtgtggcagcaatgcctggaggagcgcaacctaaaggagctgcagaagctgctaaagcaaaacttgaaggacctatggacggccttcaacgagcgctccgtggccgcgcacctggcggacattatcttccccgaacgcctgcttaaaaccctgcaacagggtctgccagacttcaccagtcaaagcatgttgcaaaactttaggaactttatcctagagcgttcaggaattctgcccgccacctgctgtgcgcttcctagcgactttgtgcccattaagtaccgtgaatgccctccgccgctttggggtcactgctaccttctgcagctagccaactaccttgcctaccactccgacatcatggaagacgtgagcggtgacggcctactggagtgtcactgtcgctgcaacctatgcaccccgcaccgctccctggtctgcaattcgcaactgcttagcgaaagtcaaattatcggtacctttgagctgcagggtccctcgcctgacgaaaagtccgcggctccggggttgaaactcactccggggctgtggacgtcggcttaccttcgcaaatttgtacctgaggactaccacgcccacgagattaggttctacgaagaccaatcccgcccgccaaatgcggagcttaccgcctgcgtcattacccagggccacatccttggccaattgcaagccatcaacaaagcccgccaagagtttctgctacgaaagggacggggggtttacctggacccccagtccggcgaggagctcaacccaatccccccgccgccgcagccctatcagcagccgcgggcccttgcttcccaggatggcacccaaaaagaagctgcagctgccgccgccgccacccacggacgaggaggaatactgggacagtcaggcagaggaggttttggacgaggaggaggagatgatggaagactgggacagcctagacgaagcttccgaggccgaagaggtgtcagacgaaacaccgtcaccctcggtcgcattcccctcgccggcgccccagaaattggcaaccgttcccagcatcgctacaacctccgctcctcaggcgccgccggcactgcctgttcgccgacccaaccgtagatgggacaccactggaaccagggccggtaagtctaagcagccgccgccgttagcccaagagcaacaacagcgccaaggctaccgctcgtggcgcgggcacaagaacgccatagttgcttgcttgcaagactgtgggggcaacatctccttcgcccgccgctttcttctctaccatcacggcgtggccttcccccgtaacatcctgcattactaccgtcatctctacagcccctactgcaccggcggcagcggcagcggcagcaacagcagcggtcacacagaagcaaaggcgaccggatagcaagactctgacaaagcccaagaaatccacagcggcggcagcagcaggaggaggagcgctgcgtctggcgcccaacgaacccgtatcgacccgcgagcttagaaataggatttttcccactctgtatgctatatttcaacaaagcaggggccaagaacaagagctgaaaataaaaaacaggtctctgcgctccctcacccgcagctgcctgtatcacaaaagcgaagatcagcttcggcgcacgctggaagacgcggaggctctcttcagcaaatactgcgcgctgactcttaaggactagtttcgcgccctttctcaaatttaagcgcgaaaactacgtcatctccagcggccacacccggcgccagcacctgtcgtcagcgccattatgagcaaggaaattcccacgccctacatgtggagttaccagccacaaatgggacttgcggctggagctgcccaagactactcaacccgaataaactacatgagcgcgggaccccacatgatatcccgggtcaacggaatccgcgcccaccgaaaccgaattctcctcgaacaggcggctattaccaccacacctcgtaataaccttaatccccgtagttggcccgctgccctggtgtaccaggaaagtcccgctcccaccactgtggtacttcccagagacgcccaggccgaagttcagatgactaactcaggggcgcagcttgcgggcggctttcgtcacagggtgcggtcgcccgggcgttttagggcggagtaacttgcatgtattgggaattgtagtttttttaaaatgggaagtgacgtatcgtgggaaaacggaagtgaagatttgaggaagttgtgggttttttggctttcgtttctgggcgtaggttcgcgtgcggttttctgggtgttttttgtggactttaaccgttacgtcattttttagtcctatatatactcgctctgtacttggccctttttacactgtgactgattgagctggtgccgtgtcgagtggtgttttttaataggtttttttactggtaaggctgactgttatggctgccgctgtggaagcgctgtatgttgttctggagcgggagggtgctattttgcctaggcaggagggtttttcaggtgtttatgtgtttttctctcctattaattttgttatacctcctatgggggctgtaatgttgtctctacgcctgcgggtatgtattcccccgggctatttcggtcgctttttagcactgaccgatgttaaccaacctgatgtgtttaccgagtcttacattatgactccggacatgaccgaggaactgtcggtggtgctttttaatcacggtgaccagtttttttacggtcacgccggcatggccgtagtccgtcttatgcttataagggttgtttttcctgttgtaagacaggcttctaatgtttaaatgtttttttttttgttattttattttgtgtttaatgcaggaacccgcagacatgtttgagagaaaaatggtgtctttttctgtggtggttccggaacttacctgcctttatctgcatgagcatgactacgatgtgcttgcttttttgcgcgaggctttgcctgattttttgagcagcaccttgcattttatatcgccgcccatgcaacaagcttacataggggctacgctggttagcatagctccgagtatgcgtgtcataatcagtgtgggttcttttgtcatggttcctggcggggaagtggccgcgctggtccgtgcagacctgcacgattatgttcagctggccctgcgaagggacctacgggatcgcggtatttttgttaatgttccgcttttgaatcttatacaggtctgtgaggaacctgaatttttgcaatcatgattcgctgcttgaggctgaaggtggagggcgctctggagcagatttttacaatggccggacttaatattcgggatttgcttagagacatattgataaggtggcgagatgaaaattatttgggcatggttgaaggtgctggaatgtttatagaggagattcaccctgaagggtttagcctttacgtccacttggacgtgagggcagtttgccttttggaagccattgtgcaacatcttacaaatgccattatctgttctttggctgtagagtttgaccacgccaccggaggggagcgcgttcacttaatagatcttcattttgaggttttggataatcttttggaataaaaaaaaaaaaacatggttcttccagctcttcccgctcctcccgtgtgtgactcgcagaacgaatgtgtaggttggctgggtgtggcttattctgcggtggtggatgttatcagggcagcggcgcatgaaggagtttacatagaacccgaagccagggggcgcctggatgctttgagagagtggatatactacaactactacacagagcgagctaagcgacgagaccggagacgcagatctgtttgtcacgcccgcacctggttttgcttcaggaaatatgactacgtccggcgttccatttggcatgacactacgaccaacacgatctcggttgtctcggcgcactccgtacagtagggatcgcctacctccttttgagacagagacccgcgctaccatactggaggatcatccgctgctgcccgaatgtaacactttgacaatgcacaacgtgagttacgtgcgaggtcttccctgcagtgtgggatttacgctgattcaggaatgggttgttccctgggatatggttctgacgcgggaggagcttgtaatcctgaggaagtgtatgcacgtgtgcctgtgttgtgccaacattgatatcatgacgagcatgatgatccatggttacgagtcctgggctctccactgtcattgttccagtcccggttccctgcagtgcatagccggcgggcaggttttggccagctggtttaggatggtggtggatggcgccatgtttaatcagaggtttatatggtaccgggaggtggtgaattacaacatgccaaaagaggtaatgtttatgtccagcgtgtttatgaggggtcgccacttaatctacctgcgcttgtggtatgatggccacgtgggttctgtggtccccgccatgagctttggatacagcgccttgcactgtgggattttgaacaatattgtggtgctgtgctgcagttactgtgctgatttaagtgagatcagggtgcgctgctgtgcccggaggacaaggcgtctcatgctgcgggcggtgcgaatcatcgctgaggagaccactgccatgttgtattcctgcaggacggagcggcggcggcagcagtttattcgcgcgctgctgcagcaccaccgccctatcctgatgcacgattatgactctacccccatgtaggcgtggacttccccttcgccgcccgttgagcaaccgcaagttggacagcagcctgtggctcagcagctggacagcgacatgaacttaagcgagctgcccggggagtttattaatatcactgatgagcgtttggctcgacaggaaaccgtgtggaatataacacctaagaatatgtctgttacccatgatatgatgctttttaaggccagccggggagaaaggactgtgtactctgtgtgttgggagggaggtggcaggttgaatactagggttctgtgagtttgattaaggtacggtgatcaatataagctatgtggtggtggggctatactactgaatgaaaaatgacttgaaattttctgcaattgaaaaataaacacgttgaaacataacatgcaacaggttcacgattctttattcctgggcaatgtaggagaaggtgtaagagttggtagcaaaagtttcagtggtgtattttccactttcccaggaccatgtaaaagacatagagtaagtgcttacctcgctagtttctgtggattcactagaatcgatgtaggatgttgcccctcctgacgcggtaggagaaggggagggtgccctgcatgtctgccgctgctcttgctcttgccgctgctgaggaggggggcgcatctgccgcagcaccggatgcatctgggaaaagcaaaaaaggggctcgtccctgtttccggaggaatttgcaagcggggtcttgcatgacggggaggcaaacccccgttcgccgcagtccggccggcccgagactcgaaccgggggtcctgcgactcaacccttggaaaataaccctccggctacagggagcgagccacttaatgctttcgctttccagcctaaccgcttacgccgcgcgcggccagtggccaaaaaagctagcgcagcagccgccgcgcctggaaggaagccaaaaggagcgctcccccgttgtctgacgtcgcacacctgggttcgacacgcgggcggtaaccgcatggatcacggcggacggccggatccggggttcgaaccccggtcgtccgccatgatacccttgcgaatttatccaccagaccacggaagagtgcccgcttacaggctctccttttgcacggtctagagcgtcaacgactgcgcacgcctcaccggccagagcgtcccgaccatggagcactttttgccgctgcgcaacatctggaaccgcgtccgcgactttccgcgcgcctccaccaccgccgccggcatcacctggatgtccaggtacatctacggattacgtcgacgtttaaaccatatgatcagctcactcaaaggcggtaatacggttatccacagaatcaggggataacgcaggaaagaacatgtgagcaaaaggccagcaaaaggccaggaaccgtaaaaaggccgcgttgctggcgtttttccataggctccgcccccctgacgagcatcacaaaaatcgacgctcaagtcagaggtggcgaaacccgacaggactataaagataccaggcgtttccccctggaagctccctcgtgcgctctcctgttccgaccctgccgcttaccggatacctgtccgcctttctcccttcgggaagcgtggcgctttctcatagctcacgctgtaggtatctcagttcggtgtaggtcgttcgctccaagctgggctgtgtgcacgaaccccccgttcagcccgaccgctgcgccttatccggtaactatcgtcttgagtccaacccggtaagacacgacttatcgccactggcagcagccactggtaacaggattagcagagcgaggtatgtaggcggtgctacagagttcttgaagtggtggcctaactacggctacactagaagaacagtatttggtatctgcgctctgctgaagccagttaccttcggaaaaagagttggtagctcttgatccggcaaacaaaccaccgctggtagcggtggtttttttgtttgcaagcagcagattacgcgcagaaaaaaaggatctcaagaagatcctttgatcttttctacggggtctgacgctcagtggaacgaaaactcacgttaagggattttggtcatgagattatcaaaaaggatcttcacctagatccttttaaattaaaaatgaagttttaaatcaatctaaagtatatatgagtaaacttggtctgacagttaccaatgcttaatcagtgaggcacctatctcagcgatctgtctatttcgttcatccatagttgcctgactccccgtcgtgtagataactacgatacgggagggcttaccatctggccccagtgctgcaatgataccgcgagacccacgctcaccggctccagatttatcagcaataaaccagccagccggaagggccgagcgcagaagtggtcctgcaactttatccgcctccatccagtctattaattgttgccgggaagctagagtaagtagttcgccagttaatagtttgcgcaacgttgttgccattgctacaggcatcgtggtgtcacgctcgtcgtttggtatggcttcattcagctccggttcccaacgatcaaggcgagttacatgatcccccatgttgtgcaaaaaagcggttagctccttcggtcctccgatcgttgtcagaagtaagttggccgcagtgttatcactcatggttatggcagcactgcataattctcttactgtcatgccatccgtaagatgcttttctgtgactggtgagtactcaaccaagtcattctgagaatagtgtatgcggcgaccgagttgctcttgcccggcgtcaatacgggataataccgcgccacatagcagaactttaaaagtgctcatcattggaaaacgttcttcggggcgaaaactctcaaggatcttaccgctgttgagatccagttcgatgtaacccactcgtgcacccaactgatcttcagcatcttttactttcaccagcgtttctgggtgagcaaaaacaggaaggcaaaatgccgcaaaaaagggaataagggcgacacggaaatgttgaatactcatactcttcctttttcaatattattgaagcatttatcagggttattgtctcatgagcggatacatatttgaatgtatttagaaaaataaacaaataggggttccgcgcacatttccccgaaaagtgccacctaaattgtaagcgttaatattttgttaaaattcgcgttaaatttttgttaaatcagctcattttttaaccaataggccgaaatcggcaaaatcccttataaatcaaaagaatagaccgagatagggttgagtgttgttccagtttggaacaagagtccactattaaagaacgtggactccaacgtcaaagggcgaaaaaccgtctatcagggcgatggcccactacgtgaaccatcaccctaatcaagttttttggggtcgaggtgccgtaaagcactaaatcggaaccctaaagggagcccccgatttagagcttgacggggaaagccggcgaacgtggcgagaaaggaagggaagaaagcgaaaggagcgggcgctagggcgctggcaagtgtagcggtcacgctgcgcgtaaccaccacacccgccgcgcttaatgcgccgctacagggcgcgatggatcc